European Patent Specification EP 3 670 661 B1, published November 1, 2023. Title: A microorganism for producing a Mycosporine-like amino acid and a method for preparing a Mycosporine-like amino acid using the same. Applicant: CJ CHEILJEDANG CORPORATION. The sequence listing filed with the application follows.

SEQUENCE LISTING (104 sequences)

SEQ ID NO: 1 - DNA, 6461 bp, Anabaena variabilis ATCC29413
atgagtatcgtccaagcaaagtttgaagctaaggaaacatcttttcatgtagaaggttacgaaaagattgagtatgatttggtgtatgtagatggtatttttgaaatccagaattctgcactagcagatgtatatcaaggttttggacgatgcttggcgattgtagatgctaacgtcagtcggttgtatggtaatcaaattcaggcatatttccagtattatggtatagaactgaggctatttcctattaccattactgaaccagataagactattcaaactttcgagagagttatagatgtctttgcagatttcaaattagtccgcaaagaaccagtattagtcgtgggtggcggtttaattacagatgttgtcggctttgcttgttctacatatcgtcgcagcagcaattacatccgcattcctactacattgattggattaattgatgccagtgtagcaattaaggtagcagttaatcatcgcaaactgaaaaaccgtttgggtgcttatcatgcttctcgcaaagtatttttagatttctccttgttgcgtactctccctacagaccaagtacgtaacgggatggcggaattggtaaaaatcgctgtagtagcgcatcaagaagtttttgaattgttggagaagtacggcgaagaattactacgtactcattttggcaatatagatgcaactccagagattaaagaaatagcccatcgtttgacttacaaagctatccataagatgttggaattggaagttcccaacctgcatgagttagacctagatagggtgattgcttacggtcacacttggagtcccaccttggaacttgcgcctcgtctacccatgttccacggacacgccgttaatgtagatatggctttctcggcaacgatcgccgcccgtagaggatatattacaattgcagaacgcgatcgtattttaggattaatgagtcgcgttggtctatccctcgaccatcccatgttggatatagatattttgtggcgtggtactgaatctatcacattaactcgtgatggtttgttaagagctgctatgccaaaacccattggtgattgtgtcttcgtcaatgacctgacaagagaagaattagcagccgcattagctgaccacaaagaactttgtaccagttatccccgtggtggtgaaggtgtggatgtgtatcccgtttatcaaaaagaattaatcgggagtgttaaataatgacttttttgaattcaaaatgcaaaatactccacggatacactgcgcgagcgcggtagcatttctgttcgcggagcgtcccgtagggaaagagaaggctacgcaaataatcggacactaattgtctttaattttgaattttgaattttgaattttgaattggagcgaagcgacttgacaaatgtgattgtccaaccaacagctagacctgttacaccattgggaattttaaccaagcagttagaagccatagtccaagaggttaagcaacatccagatttacctggggaattgatagcaaacatccatcaggcttggcgtttagccgcaggtatagacccttatttggaagaatgcaccactccagaatctcctgaactcgctgcattggcaaaaaccacagccaccgaagcctggggagaacacttccacggaggtacaaccgtccgtcctctagaacaagagatgctttctggtcatatcgaaggacaaaccttaaagatgtttgttcacatgaccaaagctaaaaaagtcttagaaattgggatgtttaccggttattcggcgctggcgatggcggaagcattaccagaggatggactgcttgtggcttgtgaagttgacccttacgcggcggaaattggacagaaagcctttcaacaatctccccacggtggaaagattcgtgtggaattggatgcagccttagcaactcttgataagttagcagaagctggggagtcttttgacttggtatttatcgacgcagataaaaaagagtatgtagcctattttcacaagttgctaggtagcagtttgttagcaccagatggctttatttgtgtagataacaccttattacaaggggaagtttatctaccagcagaggaacgtagcgtcaatggtgaagcgatcgcgcaatttaatcatacagtagctatagacccccgtgtagaacaggttttgttgccgttgcgagatggtttaacaattatccgcagaatacaaccttaattgtccaatcgactatggcacaatcccttcccctttcttccgcacctgctacaccgtctcttccttcccagacgaaaatagccgcaattatccaaaatatctgcactttggctttgttattactagcattgcccattaatgccaccattgtttttatatccttgttagtcttccgaccgcaaaaggtcaaagcagcaaacccccaaaccattcttatcagtggcggtaagatgaccaaagctttacaactagcaaggtcattccacgcggctggacatagagttgtcttggtggaaacccataaatactggttgactggtcatcgtttttcccaagcagtggataagttttacacagtccccgcaccccaggacaatccccaagcttacattcaggctttggtagatatcgtcaaacaagaaaacatcgatgtttatattcccgtcaccagtccagtgggtagctactacgactcattagccaaaccagagttatcccattattgcgaagtgtttcactttgacgcagatattacccaaatgttggatgataaatttgcgttgacacaaaaagcgcgatcgcttggtttatcagtacccaaatcctttaaaattacctcaccagaacaagtcatcaacttcgatttttctggagagacacgtaaatacatcctcaaaagcattccctacgactcagtgcggcggttggacttaaccaaactcccctgtgctactccagaggaaacagcagcattcgtcagaagtttgccaattactcccgaaaaaccgtggattatgcaggaatttatccccggtaaggaattctgcacccatagcaccgttcggaatggggaactcagactgcattgctgttgcgaatcttcagccttccaagttaattatgagaatgtaaataacccgcaaattaccgaatgggtacagcattttgtcaaggaactgaaactgacaggacagatttcctttgactttatccaagccgaagacggaacagtttacgccatcgagtgtaacccccgcacacattcagcaattaccacattttacgaccacccccaggtagcagaagcgtacttgagtcaagcaccgacgactgaaaccatacaaccactaacgacaagcaagcctacctattggacttatcacgaagtttggcgtttaactggtatccgttctttcacccagttgcaaagatggctggggaatatttggcgcgggactgatgcgatttatcagccagatgaccccttaccgtttttgatggtacatcattggcaaattcccctactgttattgaataatttgcgtcgtcttaaaggttggacgcggatagatttcaatattgggaagttggtggaattggggggagattagtttttaaacgcagagggacgctgaggttagcgcagcgaaaagttctggaggagggtttccctccgtaggaaacttttcaagagagagggacgcggagtgtgttttctctgcgtctctgcgtgagaaattttttattattgagcaaagttagaagatatgcagactatagattttaatattcgtaagttacttgtagagtggaacgcgacccacagagattatgatctttcccagagtttacatgaactaattgtagctcaagtagaacgaacacctgaggcgatcgctgtcacctttgacaagcaacaactaacttatcaagaactaaatcataaagcaaaccagctaggacattatttacaaacattaggagtccagccagaaaccctggtaggcgtttgtttagaacgttccttagaaatggttatctgtcttttaggaatcctcaaagctgggggtgcttatgttcctattgaccctgaatatcctcaagaacgcatagcttatatgctagaagattctcaggtgaaggtactactaactcaagaaaaattactcaatcaaattccccaccatcaagcacaaactatctgtgtagatagggaatgggagaaaatttccacacaagctaataccaatcccaaaagtaatataaaaacggataatcttgcttatgtaatttacacctctggttccactggtaaaccaaaaggtgcaatgaacacccacaaaggtatctgtaatcgcttattgtggatgcaggaagcttatcaaatcgattccacagatagcattttacaaaaaaccccctttagttttgatgtttccgtttgggagttcttttggactttattaactggcgcacgtttggtaatagccaaaccaggcggacataaagatagtgcttacctcatcgatttaattactcaagaacaaatcactacgttgcattttgtcccctcaatgctgcaagtgtttttacaaaatcgccatgtaagcaaatgcagctctctaaaaagagttatttgtagcggtgaagctttatctatagatttacaaaatagatttttccagcatttgcaatgtgaattacataacctctatggcccgacagaagcagcaattgatgtcacattttggcaatgtagaaaagatagtaatttaaagagtgtacctattggtcgtcccattgctaatactcaaatttatattcttgatgccgatttacaaccagtaaatattggtgtcactggtgaaatttatattggtggtgtaggggttgctcgtggttatttgaataaagaagaattgaccaaagaaaaatttattattaatccctttcccaattctgagtttaagcgactttataaaacaggtgatttagctcgttatttacccgatggaaatattgaatatcttggtagaacagattatcaagtaaaaattcggggttatagaattgaaattggcgagattgaaaatgttttatcttcacacccacaagtcagagaagctgtagtcatagcgcgggatgataacgctcaagaaaaacaaatcatcgcttatattacctataactccatcaaacctcagcttgataatctgcgtgatttcctaaaagcaaggctacctgattttatgattccagccgcttttgtgatgctggagcatcttcctttaactcccagtggtaaagtagaccgtaaggcattacctaagcctgatttatttaattatagtgaacataattcctatgtagcgcctcggaatgaagttgaagaaaaattagtacaaatctggtcgaatattctgcatttacctaaagtaggtgtgacagaaaactttttcgctattggtggtaattccctcaaagctctacatttaatttctcaaattgaagagttatttgctaaagagatatccttagcaacacttttaacaaatccagtaattgcagatttagccaaggttattcaagcaaacaaccaaatccataattcacccctagttccaattcaaccacaaggtaagcagcagcctttcttttgtatacatcctgctggtggtcatgttttatgctattttaaactcgcacaatatataggaactgaccaaccattttatggcttacaagctcaaggattttatggagatgaagcacccttgacgcgagttgaagatatggctagtctctacgtcaaaactattagagaatttcaaccccaagggccttatcgtgtcggggggtggtcatttggtggagtcgtagcttatgaagtagcacagcagttacatagacaaggacaagaagtatctttactagcaatattagattcttacgtaccgattctgctggataaacaaaaacccattgatgacgtttatttagttggtgttctctccagagtttttggcggtatgtttggtcaagataatctagtcacacctgaagaaatagaaaatttaactgtagaagaaaaaattaattacatcattgataaagcacggagcgctagaatattcccgcctggtgtagaacgtcaaaataatcgccgtattcttgatgttttggtgggaactttaaaagcaacttattcctatataagacaaccatatccaggaaaagtcactgtatttcgagccagggaaaaacatattatggctcctgacccgaccttagtttgggtagaattattttctgtaatggcggctcaagaaattaagattattgatgtccctggaaaccattattcgtttgttctagaaccccatgtacaggttttagcacagcgtttacaagattgtctggaaaataattcataa

SEQ ID NO: 2 - protein, 2035 aa, Anabaena variabilis ATCC29413
MSIVQAKFEAKETSFHVEGYEKIEYDLVYVDGIFEIQNSALADVYQGFGRCLAIVDANVSRLYGNQIQAYFQYYGIELRLFPITITEPDKTIQTFERVIDVFADFKLVRKEPVLVVGGGLITDVVGFACSTYRRSSNYIRIPTTLIGLIDASVAIKVAVNHRKLKNRLGAYHASRKVFLDFSLLRTLPTDQVRNGMAELVKIAVVAHQEVFELLEKYGEELLRTHFGNIDATPEIKEIAHRLTYKAIHKMLELEVPNLHELDLDRVIAYGHTWSPTLELAPRLPMFHGHAVNVDMAFSATIAARRGYITIAERDRILGLMSRVGLSLDHPMLDIDILWRGTESITLTRDGLLRAAMPKPIGDCVFVNDLTREELAAALADHKELCTSYPRGGEGVDVYPVYQKELIGSVKLTNVIVQPTARPVTPLGILTKQLEAIVQEVKQHPDLPGELIANIHQAWRLAAGIDPYLEECTTPESPELAALAKTTATEAWGEHFHGGTTVRPLEQEMLSGHIEGQTLKMFVHMTKAKKVLEIGMFTGYSALAMAEALPEDGLLVACEVDPYAAEIGQKAFQQSPHGGKIRVELDAALATLDKLAEAGESFDLVFIDADKKEYVAYFHKLLGSSLLAPDGFICVDNTLLQGEVYLPAEERSVNGEAIAQFNHTVAIDPRVEQVLLPLRDGLTIIRRIQPMAQSLPLSSAPATPSLPSQTKIAAIIQNICTLALLLLALPINATIVFISLLVFRPQKVKAANPQTILISGGKMTKALQLARSFHAAGHRVVLVETHKYWLTGHRFSQAVDKFYTVPAPQDNPQAYIQALVDIVKQENIDVYIPVTSPVGSYYDSLAKPELSHYCEVFHFDADITQMLDDKFALTQKARSLGLSVPKSFKITSPEQVINFDFSGETRKYILKSIPYDSVRRLDLTKLPCATPEETAAFVRSLPITPEKPWIMQEFIPGKEFCTHSTVRNGELRLHCCCESSAFQVNYENVNNPQITEWVQHFVKELKLTGQISFDFIQAEDGTVYAIECNPRTHSAITTFYDHPQVAEAYLSQAPTTETIQPLTTSKPTYWTYHEVWRLTGIRSFTQLQRWLGNIWRGTDAIYQPDDPLPFLMVHHWQIPLLLLNNLRRLKGWTRIDFNIGKLVELGGDMQTIDFNIRKLLVEWNATHRDYDLSQSLHELIVAQVERTPEAIAVTFDKQQLTYQELNHKANQLGHYLQTLGVQPETLVGVCLERSLEMVICLLGILKAGGAYVPIDPEYPQERIAYMLEDSQVKVLLTQEKLLNQIPHHQAQTICVDREWEKISTQANTNPKSNIKTDNLAYVIYTSGSTGKPKGAMNTHKGICNRLLWMQEAYQIDSTDSILQKTPFSFDVSVWEFFWTLLTGARLVIAKPGGHKDSAYLIDLITQEQITTLHFVPSMLQVFLQNRHVSKCSSLKRVICSGEALSIDLQNRFFQHLQCELHNLYGPTEAAIDVTFWQCRKDSNLKSVPIGRPIANTQIYILDADLQPVNIGVTGEIYIGGVGVARGYLNKEELTKEKFIINPFPNSEFKRLYKTGDLARYLPDGNIEYLGRTDYQVKIRGYRIEIGEIENVLSSHPQVREAVVIARDDNAQEKQIIAYITYNSIKPQLDNLRDFLKARLPDFMIPAAFVMLEHLPLTPSGKVDRKALPKPDLFNYSEHNSYVAPRNEVEEKLVQIWSNILHLPKVGVTENFFAIGGNSLKALHLISQIEELFAKEISLATLLTNPVIADLAKVIQANNQIHNSPLVPIQPQGKQQPFFCIHPAGGHVLCYFKLAQYIGTDQPFYGLQAQGFYGDEAPLTRVEDMASLYVKTIREFQPQGPYRVGGWSFGGVVAYEVAQQLHRQGQEVSLLAILDSYVPILLDKQKPIDDVYLVGVLSRVFGGMFGQDNLVTPEEIENLTVEEKINYIIDKARSARIFPPGVERQNNRRILDVLVGTLKATYSYIRQPYPGKVTVFRAREKHIMAPDPTLVWVELFSVMAAQEIKIIDVPGNHYSFVLEPHVQVLAQRLQDCLENNS

SEQ ID NO: 3 - DNA, 4528 bp, Nostoc punctiforme ATCC29133
atgagtaatgttcaagcatcgtttgaagcaacggaagctgaattccgcgtggaaggttacgaaaaaattgagtttagtcttgtctatgtaaatggtgcatttgatatcagtaacagagaaattgcagacagctatgagaagtttggccgttgtctgactgtgattgatgctaatgtcaacagattatatggcaagcaaatcaagtcatattttagacactatggtattgatctgaccgtagttcccattgtgattactgagcctactaaaacccttgcaacctttgagaaaattgttgatgctttttctgactttggtttaatccgcaaggaaccagtattagtagtgggtggtggtttaaccactgatgtagctgggtttgcgtgtgctgcttaccgtcgtaagagtaactatattcgggttccgacaacgctgattggtctgattgatgcaggtgtagcgattaaggttgcagtcaaccatcgcaagttaaaaaatcgcttgggtgcatatcatgctcctttgaaagtcatcctcgatttctccttcttgcaaacattaccaacggctcaagttcgtaatgggatggcagagttggtcaaaattgctgttgtggcgaactctgaagtctttgaattgttgtatgaatatggcgaagagttgctttccactcactttggatatgtgaatggtacaaaggaactgaaagcgatcgcacataaactcaattacgaggcaataaaaactatgctggagttggaaactccaaacttgcatgagttagacctcgatcgcgtcattgcctacggtcacacttggagtccgaccttagaattagctccgatgataccgttgtttcacggtcatgccgtcaatatagacatggctttgtctgcaactattgcggcaagacgtggctacattacatcaggagaacgcgatcgcattttgagcttgatgagtcgtataggtttatcaatcgatcatcctctactagatggcgatttgctctggtatgctacccaatctattagcttgacgcgagacgggaaacaacgcgcagctatgcctaaacccattggtgagtgcttctttgtcaacgatttcacccgtgaagaactagatgcagctttagctgaacacaaacgtctgtgtgctacataccctcgtggtggagatggcattgacgcttacatagaaactcaagaagaatccaaactattgggagtgtgaaaacatgaccagtattttaggacgagataccgcaagaccaataacgccacatagcattctggtagcacagctacaaaaaaccctcagaatggcagaggaaagtaatattccttcagagatactgacttctctgcgccaagggttgcaattagcagcaggtttagatccctatctggatgattgcactacccctgaatcgaccgcattgacagcactagcgcagaagacaagcattgaagactggagtaaacgcttcagtgatggtgaaacagtgcgtcaattagagcaagaaatgctctcaggacatcttgaaggacaaacactaaagatgtttgtgcatatcactaaggctaaaagcatcctagaagtgggaatgttcacaggatattcagctttggcaatggcagaggcgttaccagatgatgggcgactgattgcttgtgaagtagactcctatgtggccgagtttgctcaaacttgctttcaagagtctccccacggccgcaagattgttgtagaagtggcacctgcactagagacgctgcacaagctggtggctaaaaaagaatcctttgatctgatcttcattgatgcggataaaaaggagtatatagaatacttccaaattatcttggatagccatttactagctcccgacggattaatctgtgtagataatactttgttgcaaggacaagtttacctgccatcagaacagcgtacagccaatggtgaagcgatcgctcaattcaaccgcattgtcgccgcagatcctcgtgtagagcaagttctgttacccatacgagatggtataaccctgattagacgcttggtataagcggccgcgagctcctcgagatggcacaatcaatctctttatctcttcctcaatccacaacgccatcaaagggtgtgaggctaaaaatagcagctctactgaagactatcgggactctaatactactgctgatagccttgccgcttaatgctttgatagtattgatatctctgatgtgtaggccgtttacaaaaaaacctgccgtagccactcatccccagaatatcttggtcagtggcggcaaaatgaccaaagcattgcaacttgcccgctccttccatgcagccggacacagagttattctgattgaaggtcataaatactggttatcagggcatagattctcaaattctgtgagtcgtttttatacagttcctgcaccacaagacgacccagaaggctatacccaagcgctattggaaattgtcaaacgagagaagattgacgtttatgtacccgtatgcagccctgtagctagttattacgactctttggcaaagtctgcactatcagaatattgtgaggtttttcactttgatgctgatataaccaagatgctggatgataaatttgcctttaccgatcgggcgcgatcgcttggtttatcagccccgaaatcttttaaaattaccgatcctgaacaagttatcaacttcgattttagtaaagagacgcgcaaatatattcttaagagtatttcttacgactcagttcgccgcttaaatttaaccaaacttccttgtgataccccagaagagacagcagcgtttgtcaagagtttacccatcagcccagaaaaaccttggattatgcaagaatttattcctgggaaagaattatgcacccatagcacagtccgagacggcgaattaaggttgcattgctgttcaaattcttcagcgtttcagattaactatgaaaatgtcgaaaatccccaaattcaagaatgggtacaacatttcgtcaaaagtttacggctgactggacaaatatctcttgactttatccaagctgaagatggtacagcttatgccattgaatgtaatcctcgcacccattcggcgatcacaatgttctacaatcacccaggtgttgcagaagcctatcttggtaaaactcctctagctgcacctttggaacctcttgcagatagcaagcccacttactggatatatcacgaaatctggcgattgactgggattcgctctggacaacaattacaaacttggtttgggagattagtcagaggtacagatgccatttatcgcctggacgatccgataccatttttaactttgcaccattggcagattactttacttttgctacaaaatttgcaacgactcaaaggttgggtaaagatcgattttaatatcggtaaactcgtggaattagggggcgactaaaaacatgccagtacttaatatccttcatttagttgggtctgcacacgataagttttactgtgatttatcacgtctttatgcccaagactgtttagctgcaacagcagatccatcgctttataactttcaaattgcatatatcacacccgatcggcagtggcgatttcctgactctctcagtcgagaagatattgctcttaccaaaccgattcctgtgtttgatgccatacaatttctaacaggccaaaacattgacatgatgttaccacaaatgttttgtattcctggaatgactcagtaccgtgccctattcgatctgctcaagatcccttatataggaaataccccagatattatggcgatcgcggcccacaaagccagagccaaagcaattgtcgaagcagcaggggtaaaagtgcctcgtggagaattgcttcgccaaggagatattccaacaattacacctccagcagtcgtcaaacctgtaagttctgacaactctttaggagtagtcttagttaaagatgtgactgaatatgatgctgccttaaagaaagcatttgaatatgcttcggaggtcatcgtagaagcattcatcgaacttggtcgagaagtcagatgcggcatcattgtaaaagacggtgagctaataggtttaccccttgaagagtatctggtagacccacacgataaacctatccgtaactatgctgataaactccaacaaactgacgatggcgacttgcatttgactgctaaagataatatcaaggcttggattttagaccctaacgacccaatcacccaaaaggttcagcaagtggctaaaaggtgtcatcaggctttgggttgtcgccactacagtttatttgacttccgaatcgatccaaagggacaaccttggttcttagaagctggattatattgttcttttgcccccaaaagtgtgatttcttctatggcgaaagcagccggaatccctctaaatgatttattaataaccgctattaatgaaacattgggtagtaataaaaaggtgttacaaaattga

SEQ ID NO: 4 - protein, 1496 aa, Nostoc punctiforme ATCC29133
MSNVQASFEATEAEFRVEGYEKIEFSLVYVNGAFDISNREIADSYEKFGRCLTVIDANVNRLYGKQIKSYFRHYGIDLTVVPIVITEPTKTLATFEKIVDAFSDFGLIRKEPVLVVGGGLTTDVAGFACAAYRRKSNYIRVPTTLIGLIDAGVAIKVAVNHRKLKNRLGAYHAPLKVILDFSFLQTLPTAQVRNGMAELVKIAVVANSEVFELLYEYGEELLSTHFGYVNGTKELKAIAHKLNYEAIKTMLELETPNLHELDLDRVIAYGHTWSPTLELAPMIPLFHGHAVNIDMALSATIAARRGYITSGERDRILSLMSRIGLSIDHPLLDGDLLWYATQSISLTRDGKQRAAMPKPIGECFFVNDFTREELDAALAEHKRLCATYPRGGDGIDAYIETQEESKLLGVMTSILGRDTARPITPHSILVAQLQKTLRMAEESNIPSEILTSLRQGLQLAAGLDPYLDDCTTPESTALTALAQKTSIEDWSKRFSDGETVRQLEQEMLSGHLEGQTLKMFVHITKAKSILEVGMFTGYSALAMAEALPDDGRLIACEVDSYVAEFAQTCFQESPHGRKIVVEVAPALETLHKLVAKKESFDLIFIDADKKEYIEYFQIILDSHLLAPDGLICVDNTLLQGQVYLPSEQRTANGEAIAQFNRIVAADPRVEQVLLPIRDGITLIRRLVMAQSISLSLPQSTTPSKGVRLKIAALLKTIGTLILLLIALPLNALIVLISLMCRPFTKKPAVATHPQNILVSGGKMTKALQLARSFHAAGHRVILIEGHKYWLSGHRFSNSVSRFYTVPAPQDDPEGYTQALLEIVKREKIDVYVPVCSPVASYYDSLAKSALSEYCEVFHFDADITKMLDDKFAFTDRARSLGLSAPKSFKITDPEQVINFDFSKETRKYILKSISYDSVRRLNLTKLPCDTPEETAAFVKSLPISPEKPWIMQEFIPGKELCTHSTVRDGELRLHCCSNSSAFQINYENVENPQIQEWVQHFVKSLRLTGQISLDFIQAEDGTAYAIECNPRTHSAITMFYNHPGVAEAYLGKTPLAAPLEPLADSKPTYWIYHEIWRLTGIRSGQQLQTWFGRLVRGTDAIYRLDDPIPFLTLHHWQITLLLLQNLQRLKGWVKIDFNIGKLVELGGDMPVLNILHLVGSAHDKFYCDLSRLYAQDCLAATADPSLYNFQIAYITPDRQWRFPDSLSREDIALTKPIPVFDAIQFLTGQNIDMMLPQMFCIPGMTQYRALFDLLKIPYIGNTPDIMAIAAHKARAKAIVEAAGVKVPRGELLRQGDIPTITPPAVVKPVSSDNSLGVVLVKDVTEYDAALKKAFEYASEVIVEAFIELGREVRCGIIVKDGELIGLPLEEYLVDPHDKPIRNYADKLQQTDDGDLHLTAKDNIKAWILDPNDPITQKVQQVAKRCHQALGCRHYSLFDFRIDPKGQPWFLEAGLYCSFAPKSVISSMAKAAGIPLNDLLITAINETLGSNKKVLQN

SEQ ID NO: 5 - DNA, 45 bp, Artificial Sequence
  forword primer for Ava_ABCD
acaatttcacacaggaaagatatcatgagtatcgtccaagcaaag

SEQ ID NO: 6 - DNA, 45 bp, Artificial Sequence
  reverse primer for Ava_ABCD
ctcatccgccaaaacagctctagattatgaattattttccagaca

SEQ ID NO: 7 - DNA, 31 bp, Artificial Sequence
  forword primer for Npr_ABCD
gatcgatatcatgagtaatgttcaagcatcg

SEQ ID NO: 8 - DNA, 36 bp, Artificial Sequence
  reverse primer for Npr_ABCD
gatctctagatcaattttgtaacacctttttattac

SEQ ID NO: 9 - DNA, 71 bp, Artificial Sequence
  forward primer for aroD deletion cassette
tcatggggttcggtgcctgacaggctgaccgcgtgcagaaagggtaaaaagctggagctgcttcgaagttc

SEQ ID NO: 10 - DNA, 79 bp, Artificial Sequence
  reverse primer for aroD deletion cassette
atatattttttagttcggcggggagggtgttcccgccgaaatattattgcgccatggtccatatgaatatcctccttag

SEQ ID NO: 11 - DNA, 23 bp, Artificial Sequence
  forward primer for aroD deletion
caaagatttccctctggaatatg

SEQ ID NO: 12 - DNA, 21 bp, Artificial Sequence
  reverse primer for aroD deletion
cagatgtgattttccctacgc

SEQ ID NO: 13 - DNA, 40 bp, Artificial Sequence
  forward primer for aroG
aaggagctcactagtggtacggatgctcctgttatggtcg

SEQ ID NO: 14 - DNA, 41 bp, Artificial Sequence
  reverse primer for aroG
ctctcttcgacaatttccacttacccgcgacgcgcttttac

SEQ ID NO: 15 - DNA, 41 bp, Artificial Sequence
  forward primer for ppsA
gtaaaagcgcgtcgcgggtaagtggaaattgtcgaagagag

SEQ ID NO: 16 - DNA, 42 bp, Artificial Sequence
  reverse primer for ppsA
gccctagtggatctgatgggttatttcttcagttcagccagg

SEQ ID NO: 17 - DNA, 42 bp, Artificial Sequence
  forward primer for tktA
cctggctgaactgaagaaataacccatcagatccactagggc

SEQ ID NO: 18 - DNA, 42 bp, Artificial Sequence
  reverse primer for tktA
cgacaccggtcagcagggtgttacagcagttcttttgctttc

SEQ ID NO: 19 - DNA, 20 bp, Artificial Sequence
  forward primer for confirmtion of pSKH130-deltafhuA-Pn-aroG-Pn-ppsA-Pn-tktA plasmid
gaaaatgccgatgggtaccg

SEQ ID NO: 20 - DNA, 26 bp, Artificial Sequence
  reverse primer for confirmtion of pSKH130-deltafhuA-Pn-aroG-Pn-ppsA-Pn-tktA plasmid
cgttagaacgcggctacaattaatac

SEQ ID NO: 21 - DNA, 49 bp, Artificial Sequence
  forward primer for Ava_ABCD
catctcacaccgagattattttagtactatgagtatcgtccaagcaaag

SEQ ID NO: 22 - DNA, 46 bp, Artificial Sequence
  reverse primer for Ava_ABCD
caatttcgtatagagtctcactagtaccgcaaaaaggccatccgtc

SEQ ID NO: 23 - DNA, 43 bp, Artificial Sequence
  forward primer for Ptrc prompter fragment
tctcacaccgagattattttagtcgactgcacggtgcaccaat

SEQ ID NO: 24 - DNA, 50 bp, Artificial Sequence
  reverse primer for Ptrc prompter fragment
tttgcttggacgatactcatagtctgtttcctgtgtgaaattgttatccg

SEQ ID NO: 25 - DNA, 43 bp, Artificial Sequence
  forward primer for PCJ1 or PCJ2.2 prompter fragment
tctcacaccgagattattttagtcaccgcgggcttattccatt

SEQ ID NO: 26 - DNA, 49 bp, Artificial Sequence
  reverse primer for PCJ1 or PCJ2.2 prompter fragment
ttgcttggacgatactcatagtatcttaatctcctagattgggtttcac

SEQ ID NO: 27 - DNA, 50 bp, Artificial Sequence
  reverse primer for PCJ2.2 prompter fragment
tttgcttggacgatactcatagtatcttaatctcctagatttggtttcac

SEQ ID NO: 28 - DNA, 22 bp, Artificial Sequence
  forward primer for confirmation of Ava-ABCD integration
cagaatgagtgaacaaccacgg

SEQ ID NO: 29 - DNA, 25 bp, Artificial Sequence
  reverse primer for confirmation of Ava-ABCD integration
catatccaataacccagacaaaacc

SEQ ID NO: 30 - DNA, 31 bp, Artificial Sequence
  forward primer for Ptrc/PCJ1-Ava_AB or Ptrc/PCJ1-Ava_ABC
gatcggatccatgagtatcgtccaagcaaag

SEQ ID NO: 31 - DNA, 29 bp, Artificial Sequence
  reverse primer for Ptrc/PCJ1-Ava_AB
gatcactagtttaaggttgtattctgcgg

SEQ ID NO: 32 - DNA, 29 bp, Artificial Sequence
  reverse primer for Ptrc/PCJ1-Ava_ABC
gatcactagtctaatctccccccaattcc

SEQ ID NO: 33 - DNA, 60 bp, Artificial Sequence
  forward primer for Ava_ABCD
ccaaacaccaacaaaaggctctacccatatgatgagtatcgtccaagcaaagtttgaagc

SEQ ID NO: 34 - DNA, 60 bp, Artificial Sequence
  reverse primer for Ava_ABCD
agagggtgacgctagtcagaactagtttatgaattattttccagacaatcttgtaaacgc

SEQ ID NO: 35 - DNA, 58 bp, Artificial Sequence
  forward primer for CJ7 promoter fragment
ccaaacaccaacaaaaggctctacccatatgagaaacatcccagcgctactaataggg

SEQ ID NO: 36 - DNA, 48 bp, Artificial Sequence
  reverse primer for CJ7 promoter fragment
caaactttgcttggacgatactcatagtgtttcctttcgttgggtacg

SEQ ID NO: 37 - DNA, 47 bp, Artificial Sequence
  forward primer for lysc8 promoter fragment
caccaacaaaaggctctacccatatgaacactcctctggctaggtag

SEQ ID NO: 38 - DNA, 48 bp, Artificial Sequence
  reverse primer for lysc8 promoter fragment
caaactttgcttggacgatactcatctttgtgcacctttcgatctacg

SEQ ID NO: 39 - DNA, 54 bp, Artificial Sequence
  forward primer for O2 promoter fragment
ccaaacaccaacaaaaggctctacccatatgcaataatcgtgaattttggcagc

SEQ ID NO: 40 - DNA, 53 bp, Artificial Sequence
  reverse primer for O2 promoter fragment
caaactttgcttggacgatactcattgttttgatctcctccaataatctatgc

SEQ ID NO: 41 - DNA, 32 bp, Artificial Sequence
  forward primer for aroD genes to construct pDC delta aroD
gatcggatcccactggacgtttgggtgagacc

SEQ ID NO: 42 - DNA, 37 bp, Artificial Sequence
  reverse primer for aroD genes to construct pDC delta aroD
gatcggatccactagttttaggttccatttctaattg

SEQ ID NO: 43 - DNA, 29 bp, Artificial Sequence
  forward primer for aroD genes to construct pDC delta aroD
gatcactagtatgaacgacagtattctcc

SEQ ID NO: 44 - DNA, 30 bp, Artificial Sequence
  reverse primer for aroD genes to construct pDC delta aroD
gatcaagcttgttacatcctgacgttgtgg

SEQ ID NO: 45 - DNA, 30 bp, Artificial Sequence
  forward primer for Ava_A
cgcggatccatgagtatcgtccaagcaaag

SEQ ID NO: 46 - DNA, 33 bp, Artificial Sequence
  reverse primer for Ava_A
cgcctcgagttatttaacactcccgattaattc

SEQ ID NO: 47 - DNA, 31 bp, Artificial Sequence
  forward primer for Ava_B
cgcggatccatgacaaatgtgattgtccaac

SEQ ID NO: 48 - DNA, 35 bp, Artificial Sequence
  reverse primer for Ava_B
cgcctcgagttaaggttgtattctgcggataattg

SEQ ID NO: 49 - DNA, 32 bp, Artificial Sequence
  forward primer for Ava_C
cgcggatccatggcacaatcccttcccctttc

SEQ ID NO: 50 - DNA, 31 bp, Artificial Sequence
  reverse primer for Ava_C
cgcctcgagctaatctccccccaattccacc

SEQ ID NO: 51 - DNA, 34 bp, Artificial Sequence
  forward primer for Ava_D
cgcggatccatgcagactatagattttaatattc

SEQ ID NO: 52 - DNA, 33 bp, Artificial Sequence
  reverse primer for Ava_D
cgcctcgagttatgaattattttccagacaatc

SEQ ID NO: 53 - DNA, 30 bp, Artificial Sequence
  forward primer for Npr_A
cgcggatccatgagtaatgttcaagcatcg

SEQ ID NO: 54 - DNA, 29 bp, Artificial Sequence
  reverse primer for Npr_A
cgcctcgagtcacactcccaatagtttgg

SEQ ID NO: 55 - DNA, 31 bp, Artificial Sequence
  forward primer for Npr_B
cgcggatccatgaccagtattttaggacgag

SEQ ID NO: 56 - DNA, 28 bp, Artificial Sequence
  reverse primer for Npr_B
cgcctcgagttataccaagcgtctaatc

SEQ ID NO: 57 - DNA, 32 bp, Artificial Sequence
  forward primer for Npr_C
cgcggatccatggcacaatcaatctctttatc

SEQ ID NO: 58 - DNA, 31 bp, Artificial Sequence
  reverse primer for Npr_C
cgcctcgagttagtcgccccctaattccacg

SEQ ID NO: 59 - DNA, 31 bp, Artificial Sequence
  forward primer for Npr_D
cgcggatccatgccagtacttaatatccttc

SEQ ID NO: 60 - DNA, 35 bp, Artificial Sequence
  reverse primer for Npr_D
cgcctcgagtcaattttgtaacacctttttattac

SEQ ID NO: 61 - DNA, 48 bp, Artificial Sequence
  forward primer for pGPD
acgtaagataattgtatattacgcagtttatcattatcaatactcgcc

SEQ ID NO: 62 - DNA, 40 bp, Artificial Sequence
  reverse primer for pGPD
gtaacgacaatcctctccatgtggtcttgaatcaaagctg

SEQ ID NO: 63 - DNA, 39 bp, Artificial Sequence
  forward primer for LoxP(Ura)
ccgattgtcaatcagcgtaacagctgaagcttcgtacgc

SEQ ID NO: 64 - DNA, 44 bp, Artificial Sequence
  reverse primer for LoxP(Ura)
ttgttttggccagtcggcaagggcataggccactagtggatctg

SEQ ID NO: 65 - DNA, 40 bp, Artificial Sequence
  forward primer for aroB
cagctttgattcaagaccacatggagaggattgtcgttac

SEQ ID NO: 66 - DNA, 39 bp, Artificial Sequence
  reverse primer for aroB
gcgtacgaagcttcagctgttacgctgattgacaatcgg

SEQ ID NO: 67 - DNA, 32 bp, Artificial Sequence
  forward primer for ARO1 fragment 1
accattcaagagtatatgagagaaggaaaact

SEQ ID NO: 68 - DNA, 47 bp, Artificial Sequence
  reverse primer for ARO1 fragment 1
ggcgagtattgataatgataaactgcgtaatatacaattatcttacg

SEQ ID NO: 69 - DNA, 44 bp, Artificial Sequence
  forward primer for ARO1 fragment 2
cagatccactagtggcctatgcccttgccgactggccaaaacaa

SEQ ID NO: 70 - DNA, 20 bp, Artificial Sequence
  reverse primer for ARO1 fragment 2
caaatatcaatggcacgttg

SEQ ID NO: 71 - DNA, 759 bp, Escherichia coli W3110
atgaaaaccgtaactgtaaaagatctcgtcattggtacgggcgcacctaaaatcatcgtctcgctgatggcgaaagatatcgccagcgtgaaatccgaagctctcgcctatcgtgaagcggactttgatattctggaatggcgtgtggaccactatgccgacctctccaatgtggagtctgtcatggcggcagcaaaaattctccgtgagaccatgccagaaaaaccgctgctgtttaccttccgcagtgccaaagaaggcggcgagcaggcgatttccaccgaggcttatattgcactcaatcgtgcagccatcgacagcggcctggttgatatgatcgatctggagttatttaccggtgatgatcaggttaaagaaaccgtcgcctacgcccacgcgcatgatgtgaaagtagtcatgtccaaccatgacttccataaaacgccggaagccgaagaaatcattgcccgtctgcgcaaaatgcaatccttcgacgccgatattcctaagattgcgctgatgccgcaaagtaccagcgatgtgctgacgttgcttgccgcgaccctggagatgcaggagcagtatgccgatcgtccaattatcacgatgtcgatggcaaaaactggcgtaatttctcgtctggctggtgaagtatttggctcggcggcaacttttggtgcggtaaaaaaagcgtctgcgccagggcaaatctcggtaaatgatttgcgcacggtattaactattttacaccaggcataa

SEQ ID NO: 72 - protein, 252 aa, Escherichia coli W3110
MKTVTVKDLVIGTGAPKIIVSLMAKDIASVKSEALAYREADFDILEWRVDHYADLSNVESVMAAAKILRETMPEKPLLFTFRSAKEGGEQAISTEAYIALNRAAIDSGLVDMIDLELFTGDDQVKETVAYAHAHDVKVVMSNHDFHKTPEAEEIIARLRKMQSFDADIPKIALMPQSTSDVLTLLAATLEMQEQYADRPIITMSMAKTGVISRLAGEVFGSAATFGAVKKASAPGQISVNDLRTVLTILHQA

SEQ ID NO: 73 - DNA, 1053 bp, Escherichia coli W3110
atgaattatcagaacgacgatttacgcatcaaagaaatcaaagagttacttcctcctgtcgcattgctggaaaaattccccgctactgaaaatgccgcgaatacggttgcccatgcccgaaaagcgatccataagatcctgaaaggtaatgatgatcgcctgttggttgtgattggcccatgctcaattcatgatcctgtcgcggcaaaagagtatgccactcgcttgctggcgctgcgtgaagagctgaaagatgagctggaaatcgtaatgcgcgtctattttgaaaagccgcgtaccacggtgggctggaaagggctgattaacgatccgcatatggataatagcttccagatcaacgacggtctgcgtatagcccgtaaattgctgcttgatattaacgacagcggtctgccagcggcaggtgagtttctcgatatgatcaccccacaatatctcgctgacctgatgagctggggcgcaattggcgcacgtaccaccgaatcgcaggtgcaccgcgaactggcatcagggctttcttgtccggtcggcttcaaaaatggcaccgacggtacgattaaagtggctatcgatgccattaatgccgccggtgcgccgcactgcttcctgtccgtaacgaaatgggggcattcggcgattgtgaataccagcggtaacggcgattgccatatcattctgcgcggcggtaaagagcctaactacagcgcgaagcacgttgctgaagtgaaagaagggctgaacaaagcaggcctgccagcacaggtgatgatcgatttcagccatgctaactcgtccaaacaattcaaaaagcagatggatgtttgtgctgacgtttgccagcagattgccggtggcgaaaaggccattattggcgtgatggtggaaagccatctggtggaaggcaatcagagcctcgagagcggggagccgctggcctacggtaagagcatcaccgatgcctgcatcggctgggaagataccgatgctctgttacgtcaactggcgaatgcagtaaaagcgcgtcgcgggtaa

SEQ ID NO: 74 - protein, 350 aa, Escherichia coli W3110
MNYQNDDLRIKEIKELLPPVALLEKFPATENAANTVAHARKAIHKILKGNDDRLLVVIGPCSIHDPVAAKEYATRLLALREELKDELEIVMRVYFEKPRTTVGWKGLINDPHMDNSFQINDGLRIARKLLLDINDSGLPAAGEFLDMITPQYLADLMSWGAIGARTTESQVHRELASGLSCPVGFKNGTDGTIKVAIDAINAAGAPHCFLSVTKWGHSAIVNTSGNGDCHIILRGGKEPNYSAKHVAEVKEGLNKAGLPAQVMIDFSHANSSKQFKKQMDVCADVCQQIAGGEKAIIGVMVESHLVEGNQSLESGEPLAYGKSITDACIGWEDTDALLRQLANAVKARRG

SEQ ID NO: 75 - DNA, 2379 bp, Escherichia coli W3110
atgtccaacaatggctcgtcaccgctggtgctttggtataaccaactcggcatgaatgatgtagacagggttgggggcaaaaatgcctccctgggtgaaatgattactaatctttccggaatgggtgtttccgttccgaatggtttcgccacaaccgccgacgcgtttaaccagtttctggaccaaagcggcgtaaaccagcgcatttatgaactgctggataaaacggatattgacgatgttactcagcttgcgaaagcgggcgcgcaaatccgccagtggattatcgacactcccttccagcctgagctggaaaacgccatccgcgaagcctatgcacagctttccgccgatgacgaaaacgcctcttttgcggtgcgctcctccgccaccgcagaagatatgccggacgcttcttttgccggtcagcaggaaaccttcctcaacgttcagggttttgacgccgttctcgtggcagtgaaacatgtatttgcttctctgtttaacgatcgcgccatctcttatcgtgtgcaccagggttacgatcaccgtggtgtggcgctctccgccggtgttcaacggatggtgcgctctgacctcgcatcatctggcgtgatgttctccattgataccgaatccggctttgaccaggtggtgtttatcacttccgcatggggccttggtgagatggtcgtgcagggtgcggttaacccggatgagttttacgtgcataaaccgacactggcggcgaatcgcccggctatcgtgcgccgcaccatggggtcgaaaaaaatccgcatggtttacgcgccgacccaggagcacggcaagcaggttaaaatcgaagacgtaccgcaggaacagcgtgacatcttctcgctgaccaacgaagaagtgcaggaactggcaaaacaggccgtacaaattgagaaacactacggtcgcccgatggatattgagtgggcgaaagatggccacaccggtaaactgttcattgtgcaggcgcgtccggaaaccgtgcgctcacgcggtcaggtcatggagcgttatacgctgcattcacagggtaagattatcgccgaaggccgtgctatcggtcatcgcatcggtgcgggtccggtgaaagtcatccatgacatcagcgaaatgaaccgcatcgaacctggcgacgtgctggttactgacatgaccgacccggactgggaaccgatcatgaagaaagcatctgccatcgtcaccaaccgtggcggtcgtacctgtcacgcggcgatcatcgctcgtgaactgggcattccggcggtagtgggctgtggagatgcaacagaacggatgaaagacggtgagaacgtcactgtttcttgtgccgaaggtgataccggttacgtctatgcggagttgctggaatttagcgtgaaaagctccagcgtagaaacgatgccggatctgccgttgaaagtgatgatgaacgtcggtaacccggaccgtgctttcgacttcgcctgcctaccgaacgaaggcgtgggccttgcgcgtctggaatttatcatcaaccgtatgattggcgtccacccacgcgcactgcttgagtttgacgatcaggaaccgcagttgcaaaacgaaatccgcgagatgatgaaaggttttgattctccgcgtgaattttacgttggtcgtctgactgaagggatcgcgacgctgggtgccgcgttttatccgaagcgcgtcattgtccgtctctctgattttaaatcgaacgaatatgccaacctggtcggtggtgagcgttacgagccagatgaagagaacccgatgctcggcttccgtggcgcgggccgctatgtttccgacagcttccgcgactgtttcgcgctggagtgtgaagcagtgaaacgtgtgcgcaacgacatgggactgaccaacgttgagatcatgatcccgttcgtgcgtaccgtagatcaggcgaaagcggtggttgaagaactggcgcgtcaggggctgaaacgtggcgagaacgggctgaaaatcatcatgatgtgtgaaatcccgtccaacgccttgctggccgagcagttcctcgaatatttcgacggcttctcaattggctcaaacgatatgacgcagctggcgctcggtctggaccgtgactccggcgtggtgtctgaattgttcgatgagcgcaacgatgcggtgaaagcactgctgtcgatggctatccgtgccgcgaagaaacagggcaaatatgtcgggatttgcggtcagggtccgtccgaccacgaagactttgccgcatggttgatggaagaggggatcgatagcctgtctctgaacccggacaccgtggtgcaaacctggttaagcctggctgaactgaagaaataa

SEQ ID NO: 76 - protein, 792 aa, Escherichia coli W3110
MSNNGSSPLVLWYNQLGMNDVDRVGGKNASLGEMITNLSGMGVSVPNGFATTADAFNQFLDQSGVNQRIYELLDKTDIDDVTQLAKAGAQIRQWIIDTPFQPELENAIREAYAQLSADDENASFAVRSSATAEDMPDASFAGQQETFLNVQGFDAVLVAVKHVFASLFNDRAISYRVHQGYDHRGVALSAGVQRMVRSDLASSGVMFSIDTESGFDQVVFITSAWGLGEMVVQGAVNPDEFYVHKPTLAANRPAIVRRTMGSKKIRMVYAPTQEHGKQVKIEDVPQEQRDIFSLTNEEVQELAKQAVQIEKHYGRPMDIEWAKDGHTGKLFIVQARPETVRSRGQVMERYTLHSQGKIIAEGRAIGHRIGAGPVKVIHDISEMNRIEPGDVLVTDMTDPDWEPIMKKASAIVTNRGGRTCHAAIIARELGIPAVVGCGDATERMKDGENVTVSCAEGDTGYVYAELLEFSVKSSSVETMPDLPLKVMMNVGNPDRAFDFACLPNEGVGLARLEFIINRMIGVHPRALLEFDDQEPQLQNEIREMMKGFDSPREFYVGRLTEGIATLGAAFYPKRVIVRLSDFKSNEYANLVGGERYEPDEENPMLGFRGAGRYVSDSFRDCFALECEAVKRVRNDMGLTNVEIMIPFVRTVDQAKAVVEELARQGLKRGENGLKIIMMCEIPSNALLAEQFLEYFDGFSIGSNDMTQLALGLDRDSGVVSELFDERNDAVKALLSMAIRAAKKQGKYVGICGQGPSDHEDFAAWLMEEGIDSLSLNPDTVVQTWLSLAELKK

SEQ ID NO: 77 - DNA, 1992 bp, Escherichia coli W3110
atgtcctcacgtaaagagcttgccaatgctattcgtgcgctgagcatggacgcagtacagaaagccaaatccggtcacccgggtgcccctatgggtatggctgacattgccgaagtcctgtggcgtgatttcctgaaacacaacccgcagaatccgtcctgggctgaccgtgaccgcttcgtgctgtccaacggccacggctccatgctgatctacagcctgctgcacctcaccggttacgatctgccgatggaagaactgaaaaacttccgtcagctgcactctaaaactccgggtcacccggaagtgggttacaccgctggtgtggaaaccaccaccggtccgctgggtcagggtattgccaacgcagtcggtatggcgattgcagaaaaaacgctggcggcgcagtttaaccgtccgggccacgacattgtcgaccactacacctacgccttcatgggcgacggctgcatgatggaaggcatctcccacgaagtttgctctctggcgggtacgctgaagctgggtaaactgattgcattctacgatgacaacggtatttctatcgatggtcacgttgaaggctggttcaccgacgacaccgcaatgcgtttcgaagcttacggctggcacgttattcgcgacatcgacggtcatgacgcggcatctatcaaacgcgcagtagaagaagcgcgcgcagtgactgacaaaccttccctgctgatgtgcaaaaccatcatcggtttcggttccccgaacaaagccggtacccacgactcccacggtgcgccgctgggcgacgctgaaattgccctgacccgcgaacaactgggctggaaatatgcgccgttcgaaatcccgtctgaaatctatgctcagtgggatgcgaaagaagcaggccaggcgaaagaatccgcatggaacgagaaattcgctgcttacgcgaaagcttatccgcaggaagccgctgaatttacccgccgtatgaaaggcgaaatgccgtctgacttcgacgctaaagcgaaagagttcatcgctaaactgcaggctaatccggcgaaaatcgccagccgtaaagcgtctcagaatgctatcgaagcgttcggtccgctgttgccggaattcctcggcggttctgctgacctggcgccgtctaacctgaccctgtggtctggttctaaagcaatcaacgaagatgctgcgggtaactacatccactacggtgttcgcgagttcggtatgaccgcgattgctaacggtatctccctgcacggtggcttcctgccgtacacctccaccttcctgatgttcgtggaatacgcacgtaacgccgtacgtatggctgcgctgatgaaacagcgtcaggtgatggtttacacccacgactccatcggtctgggcgaagacggcccgactcaccagccggttgagcaggtcgcttctctgcgcgtaaccccgaacatgtctacatggcgtccgtgtgaccaggttgaatccgcggtcgcgtggaaatacggtgttgagcgtcaggacggcccgaccgcactgatcctctcccgtcagaacctggcgcagcaggaacgaactgaagagcaactggcaaacatcgcgcgcggtggttatgtgctgaaagactgcgccggtcagccggaactgattttcatcgctaccggttcagaagttgaactggctgttgctgcctacgaaaaactgactgccgaaggcgtgaaagcgcgcgtggtgtccatgccgtctaccgacgcatttgacaagcaggatgctgcttaccgtgaatccgtactgccgaaagcggttactgcacgcgttgctgtagaagcgggtattgctgactactggtacaagtatgttggcctgaacggtgctatcgtcggtatgaccaccttcggtgaatctgctccggcagagctgctgtttgaagagttcggcttcactgttgataacgttgttgcgaaagcaaaagaactgctgtaa

SEQ ID NO: 78 - protein, 663 aa, Escherichia coli W3110
MSSRKELANAIRALSMDAVQKAKSGHPGAPMGMADIAEVLWRDFLKHNPQNPSWADRDRFVLSNGHGSMLIYSLLHLTGYDLPMEELKNFRQLHSKTPGHPEVGYTAGVETTTGPLGQGIANAVGMAIAEKTLAAQFNRPGHDIVDHYTYAFMGDGCMMEGISHEVCSLAGTLKLGKLIAFYDDNGISIDGHVEGWFTDDTAMRFEAYGWHVIRDIDGHDAASIKRAVEEARAVTDKPSLLMCKTIIGFGSPNKAGTHDSHGAPLGDAEIALTREQLGWKYAPFEIPSEIYAQWDAKEAGQAKESAWNEKFAAYAKAYPQEAAEFTRRMKGEMPSDFDAKAKEFIAKLQANPAKIASRKASQNAIEAFGPLLPEFLGGSADLAPSNLTLWSGSKAINEDAAGNYIHYGVREFGMTAIANGISLHGGFLPYTSTFLMFVEYARNAVRMAALMKQRQVMVYTHDSIGLGEDGPTHQPVEQVASLRVTPNMSTWRPCDQVESAVAWKYGVERQDGPTALILSRQNLAQQERTEEQLANIARGGYVLKDCAGQPELIFIATGSEVELAVAAYEKLTAEGVKARVVSMPSTDAFDKQDAAYRESVLPKAVTARVAVEAGIADYWYKYVGLNGAIVGMTTFGESAPAELLFEEFGFTVDNVVAKAKELL

SEQ ID NO: 79 - DNA, 438 bp, Corynebacterium glutamicum ATCC 13032
atgcctggaaaaattctcctcctcaacggcccaaacctgaacatgctgggcaaacgcgagcctgacatttacggacacgacaccttggaagacgtcgtcgcgctggcaaccgctgaggctgcgaagcacggccttgaggttgaggcgctgcagagcaatcacgaaggtgagctaatcgatgcgctgcacaacgctcgcggcacccacatcggttgcgtgattaaccccggcggcctgactcacacttcggtggcgcttttggatgctgtgaaggcgtctgagcttcctaccgttgaggtgcacatttccaatccgcatgcccgtgaagagttccgccaccattcttacatttccctcgccgcggtctccgttatcgctggcgctggcatccagggttaccgtttcgcggtcgatatcctggcaaatctcaaaaagtag

SEQ ID NO: 80 - protein, 145 aa, Corynebacterium glutamicum ATCC 13032
MPGKILLLNGPNLNMLGKREPDIYGHDTLEDVVALATAEAAKHGLEVEALQSNHEGELIDALHNARGTHIGCVINPGGLTHTSVALLDAVKASELPTVEVHISNPHAREEFRHHSYISLAAVSVIAGAGIQGYRFAVDILANLKK

SEQ ID NO: 81 - DNA, 4767 bp, Saccharomyces cerevisiae
atggtgcagttagccaaagtcccaattctaggaaatgatattatccacgttgggtataacattcatgaccatttggttgaaaccataattaaacattgtccttcttcgacatacgttatttgcaatgatacgaacttgagtaaagttccatactaccagcaattagtcctggaattcaaggcttctttgccagaaggctctcgtttacttacttatgttgttaaaccaggtgagacaagtaaaagtagagaaaccaaagcgcagctagaagattatcttttagtggaaggatgtactcgtgatacggttatggtagcgatcggtggtggtgttattggtgacatgattgggttcgttgcatctacatttatgagaggtgttcgtgttgtccaagtaccaacatccttattggcaatggtcgattcctccattggtggtaaaactgctattgacactcctctaggtaaaaactttattggtgcattttggcaaccaaaatttgtccttgtagatattaaatggctagaaacgttagccaagagagagtttatcaatgggatggcagaagttatcaagactgcttgtatttggaacgctgacgaatttactagattagaatcaaacgcttcgttgttcttaaatgttgttaatggggcaaaaaatgtcaaggttaccaatcaattgacaaacgagattgacgagatatcgaatacagatattgaagctatgttggatcatacatataagttagttcttgagagtattaaggtcaaagcggaagttgtctcttcggatgaacgtgaatccagtctaagaaaccttttgaacttcggacattctattggtcatgcttatgaagctatactaaccccacaagcattacatggtgaatgtgtgtccattggtatggttaaagaggcggaattatcccgttatttcggtattctctcccctacccaagttgcacgtctatccaagattttggttgcctacgggttgcctgtttcgcctgatgagaaatggtttaaagagctaaccttacataagaaaacaccattggatatcttattgaagaaaatgagtattgacaagaaaaacgagggttccaaaaagaaggtggtcattttagaaagtattggtaagtgctatggtgactccgctcaatttgttagcgatgaagacctgagatttattctaacagatgaaaccctcgtttaccccttcaaggacatccctgctgatcaacagaaagttgttatcccccctggttctaagtccatctccaatcgtgctttaattcttgctgccctcggtgaaggtcaatgtaaaatcaagaacttattacattctgatgatactaaacatatgttaaccgctgttcatgaattgaaaggtgctacgatatcatgggaagataatggtgagacggtagtggtggaaggacatggtggttccacattgtcagcttgtgctgaccccttatatctaggtaatgcaggtactgcatctagatttttgacttccttggctgccttggtcaattctacttcaagccaaaagtatatcgttttaactggtaacgcaagaatgcaacaaagaccaattgctcctttggtcgattctttgcgtgctaatggtactaaaattgagtacttgaataatgaaggttccctgccaatcaaagtttatactgattcggtattcaaaggtggtagaattgaattagctgctacagtttcttctcagtacgtatcctctatcttgatgtgtgccccatacgctgaagaacctgtaactttggctcttgttggtggtaagccaatctctaaattgtacgtcgatatgacaataaaaatgatggaaaaattcggtatcaatgttgaaacttctactacagaaccttacacttattatattccaaagggacattatattaacccatcagaatacgtcattgaaagtgatgcctcaagtgctacatacccattggccttcgccgcaatgactggtactaccgtaacggttccaaacattggttttgagtcgttacaaggtgatgccagatttgcaagagatgtcttgaaacctatgggttgtaaaataactcaaacggcaacttcaactactgtttcgggtcctcctgtaggtactttaaagccattaaaacatgttgatatggagccaatgactgatgcgttcttaactgcatgtgttgttgccgctatttcgcacgacagtgatccaaattctgcaaatacaaccaccattgaaggtattgcaaaccagcgtgtcaaagagtgtaacagaattttggccatggctacagagctcgccaaatttggcgtcaaaactacagaattaccagatggtattcaagtccatggtttaaactcgataaaagatttgaaggttccttccgactcttctggacctgtcggtgtatgcacatatgatgatcatcgtgtggccatgagtttctcgcttcttgcaggaatggtaaattctcaaaatgaacgtgacgaagttgctaatcctgtaagaatacttgaaagacattgtactggtaaaacctggcctggctggtgggatgtgttacattccgaactaggtgccaaattagatggtgcagaacctttagagtgcacatccaaaaagaactcaaagaaaagcgttgtcattattggcatgagagcagctggcaaaactactataagtaaatggtgcgcatccgctctgggttacaaattagttgacctagacgagctgtttgagcaacagcataacaatcaaagtgttaaacaatttgttgtggagaacggttgggagaagttccgtgaggaagaaacaagaattttcaaggaagttattcaaaattacggcgatgatggatatgttttctcaacaggtggcggtattgttgaaagcgctgagtctagaaaagccttaaaagattttgcctcatcaggtggatacgttttacacttacatagggatattgaggagacaattgtctttttacaaagtgatccttcaagacctgcctatgtggaagaaattcgtgaagtttggaacagaagggaggggtggtataaagaatgctcaaatttctctttctttgctcctcattgctccgcagaagctgagttccaagctctaagaagatcgtttagtaagtacattgcaaccattacaggtgtcagagaaatagaaattccaagcggaagatctgcctttgtgtgtttaacctttgatgacttaactgaacaaactgagaatttgactccaatctgttatggttgtgaggctgtagaggtcagagtagaccatttggctaattactctgctgatttcgtgagtaaacagttatctatattgcgtaaagccactgacagtattcctatcatttttactgtgcgaaccatgaagcaaggtggcaactttcctgatgaagagttcaaaaccttgagagagctatacgatattgccttgaagaatggtgttgaattccttgacttagaactaactttacctactgatatccaatatgaggttattaacaaaaggggcaacaccaagatcattggttcccatcatgacttccaaggattatactcctgggacgacgctgaatgggaaaacagattcaatcaagcgttaactcttgatgtggatgttgtaaaatttgtgggtacggctgttaatttcgaagataatttgagactggaacactttagggatacacacaagaataagcctttaattgcagttaatatgacttctaaaggtagcatttctcgtgttttgaataatgttttaacacctgtgacatcagatttattgcctaactccgctgcccctggccaattgacagtagcacaaattaacaagatgtatacatctatgggaggtatcgagcctaaggaactgtttgttgttggaaagccaattggccactctagatcgccaattttacataacactggctatgaaattttaggtttacctcacaagttcgataaatttgaaactgaatccgcacaattggtgaaagaaaaacttttggacggaaacaagaactttggcggtgctgcagtcacaattcctctgaaattagatataatgcagtacatggatgaattgactgatgctgctaaagttattggtgctgtaaacacagttataccattgggtaacaagaagtttaagggtgataataccgactggttaggtatccgtaatgccttaattaacaatggcgttcccgaatatgttggtcataccgctggtttggttatcggtgcaggtggcacttctagagccgccctttacgccttgcacagtttaggttgcaaaaagatcttcataatcaacaggacaacttcgaaattgaagccattaatagagtcacttccatctgaattcaacattattggaatagagtccactaaatctatagaagagattaaggaacacgttggcgttgctgtcagctgtgtaccagccgacaaaccattagatgacgaacttttaagtaagctggagagattccttgtgaaaggtgcccatgctgcttttgtaccaaccttattggaagccgcatacaaaccaagcgttactcccgttatgacaatttcacaagacaaatatcaatggcacgttgtccctggatcacaaatgttagtacaccaaggtgtagctcagtttgaaaagtggacaggattcaagggccctttcaaggccatttttgatgccgttacgaaagagtag

SEQ ID NO: 82 - protein, 1588 aa, Saccharomyces cerevisiae
MVQLAKVPILGNDIIHVGYNIHDHLVETIIKHCPSSTYVICNDTNLSKVPYYQQLVLEFKASLPEGSRLLTYVVKPGETSKSRETKAQLEDYLLVEGCTRDTVMVAIGGGVIGDMIGFVASTFMRGVRVVQVPTSLLAMVDSSIGGKTAIDTPLGKNFIGAFWQPKFVLVDIKWLETLAKREFINGMAEVIKTACIWNADEFTRLESNASLFLNVVNGAKNVKVTNQLTNEIDEISNTDIEAMLDHTYKLVLESIKVKAEVVSSDERESSLRNLLNFGHSIGHAYEAILTPQALHGECVSIGMVKEAELSRYFGILSPTQVARLSKILVAYGLPVSPDEKWFKELTLHKKTPLDILLKKMSIDKKNEGSKKKVVILESIGKCYGDSAQFVSDEDLRFILTDETLVYPFKDIPADQQKVVIPPGSKSISNRALILAALGEGQCKIKNLLHSDDTKHMLTAVHELKGATISWEDNGETVVVEGHGGSTLSACADPLYLGNAGTASRFLTSLAALVNSTSSQKYIVLTGNARMQQRPIAPLVDSLRANGTKIEYLNNEGSLPIKVYTDSVFKGGRIELAATVSSQYVSSILMCAPYAEEPVTLALVGGKPISKLYVDMTIKMMEKFGINVETSTTEPYTYYIPKGHYINPSEYVIESDASSATYPLAFAAMTGTTVTVPNIGFESLQGDARFARDVLKPMGCKITQTATSTTVSGPPVGTLKPLKHVDMEPMTDAFLTACVVAAISHDSDPNSANTTTIEGIANQRVKECNRILAMATELAKFGVKTTELPDGIQVHGLNSIKDLKVPSDSSGPVGVCTYDDHRVAMSFSLLAGMVNSQNERDEVANPVRILERHCTGKTWPGWWDVLHSELGAKLDGAEPLECTSKKNSKKSVVIIGMRAAGKTTISKWCASALGYKLVDLDELFEQQHNNQSVKQFVVENGWEKFREEETRIFKEVIQNYGDDGYVFSTGGGIVESAESRKALKDFASSGGYVLHLHRDIEETIVFLQSDPSRPAYVEEIREVWNRREGWYKECSNFSFFAPHCSAEAEFQALRRSFSKYIATITGVREIEIPSGRSAFVCLTFDDLTEQTENLTPICYGCEAVEVRVDHLANYSADFVSKQLSILRKATDSIPIIFTVRTMKQGGNFPDEEFKTLRELYDIALKNGVEFLDLELTLPTDIQYEVINKRGNTKIIGSHHDFQGLYSWDDAEWENRFNQALTLDVDVVKFVGTAVNFEDNLRLEHFRDTHKNKPLIAVNMTSKGSISRVLNNVLTPVTSDLLPNSAAPGQLTVAQINKMYTSMGGIEPKELFVVGKPIGHSRSPILHNTGYEILGLPHKFDKFETESAQLVKEKLLDGNKNFGGAAVTIPLKLDIMQYMDELTDAAKVIGAVNTVIPLGNKKFKGDNTDWLGIRNALINNGVPEYVGHTAGLVIGAGGTSRAALYALHSLGCKKIFIINRTTSKLKPLIESLPSEFNIIGIESTKSIEEIKEHVGVAVSCVPADKPLDDELLSKLERFLVKGAHAAFVPTLLEAAYKPSVTPVMTISQDKYQWHVVPGSQMLVHQGVAQFEKWTGFKGPFKAIFDAVTKE

SEQ ID NO: 83 - DNA, 1089 bp, Escherichia coli W3110
atggagaggattgtcgttactctcggggaacgtagttacccaattaccatcgcatctggtttgtttaatgaaccagcttcattcttaccgctgaaatcgggcgagcaggtcatgttggtcaccaacgaaaccctggctcctctgtatctcgataaggtccgcggcgtacttgaacaggcgggtgttaacgtcgatagcgttatcctccctgacggcgagcagtataaaagcctggctgtactcgataccgtctttacggcgttgttacaaaaaccgcatggtcgcgatactacgctggtggcgcttggcggcggcgtagtgggcgatctgaccggcttcgcggcggcgagttatcagcgcggtgtccgtttcattcaagtcccgacgacgttactgtcgcaggtcgattcctccgttggcggcaaaactgcggtcaaccatcccctcggtaaaaacatgattggcgcgttctaccaacctgcttcagtggtggtggatctcgactgtctgaaaacgcttcccccgcgtgagttagcgtcggggctggcagaagtcatcaaatacggcattattcttgacggtgcgttttttaactggctggaagagaatctggatgcgttgttgcgtctggacggtccggcaatggcgtactgtattcgccgttgttgtgaactgaaggcagaagttgtcgccgccgacgagcgcgaaaccgggttacgtgctttactgaatctgggacacacctttggtcatgccattgaagctgaaatggggtatggcaattggttacatggtgaagcggtcgctgcgggtatggtgatggcggcgcggacgtcggaacgtctcgggcagtttagttctgccgaaacgcagcgtattataaccctgctcaagcgggctgggttaccggtcaatgggccgcgcgaaatgtccgcgcaggcgtatttaccgcatatgctgcgtgacaagaaagtccttgcgggagagatgcgcttaattcttccgttggcaattggtaagagtgaagttcgcagcggcgtttcgcacgagcttgttcttaacgccattgccgattgtcaatcagcgtaa

SEQ ID NO: 84 - protein, 362 aa, Escherichia coli W3110
MERIVVTLGERSYPITIASGLFNEPASFLPLKSGEQVMLVTNETLAPLYLDKVRGVLEQAGVNVDSVILPDGEQYKSLAVLDTVFTALLQKPHGRDTTLVALGGGVVGDLTGFAAASYQRGVRFIQVPTTLLSQVDSSVGGKTAVNHPLGKNMIGAFYQPASVVVDLDCLKTLPPRELASGLAEVIKYGIILDGAFFNWLEENLDALLRLDGPAMAYCIRRCCELKAEVVAADERETGLRALLNLGHTFGHAIEAEMGYGNWLHGEAVAAGMVMAARTSERLGQFSSAETQRIITLLKRAGLPVNGPREMSAQAYLPHMLRDKKVLAGEMRLILPLAIGKSEVRSGVSHELVLNAIADCQSA

SEQ ID NO: 85 - DNA, 2247 bp, Anabaena variabilis ATCC29413
atgagtatcgtccaagcaaagtttgaagctaaggaaacatcttttcatgtagaaggttacgaaaagattgagtatgatttggtgtatgtagatggtatttttgaaatccagaattctgcactagcagatgtatatcaaggttttggacgatgcttggcgattgtagatgctaacgtcagtcggttgtatggtaatcaaattcaggcatatttccagtattatggtatagaactgaggctatttcctattaccattactgaaccagataagactattcaaactttcgagagagttatagatgtctttgcagatttcaaattagtccgcaaagaaccagtattagtcgtgggtggcggtttaattacagatgttgtcggctttgcttgttctacatatcgtcgcagcagcaattacatccgcattcctactacattgattggattaattgatgccagtgtagcaattaaggtagcagttaatcatcgcaaactgaaaaaccgtttgggtgcttatcatgcttctcgcaaagtatttttagatttctccttgttgcgtactctccctacagaccaagtacgtaacgggatggcggaattggtaaaaatcgctgtagtagcgcatcaagaagtttttgaattgttggagaagtacggcgaagaattactacgtactcattttggcaatatagatgcaactccagagattaaagaaatagcccatcgtttgacttacaaagctatccataagatgttggaattggaagttcccaacctgcatgagttagacctagatagggtgattgcttacggtcacacttggagtcccaccttggaacttgcgcctcgtctacccatgttccacggacacgccgttaatgtagatatggctttctcggcaacgatcgccgcccgtagaggatatattacaattgcagaacgcgatcgtattttaggattaatgagtcgcgttggtctatccctcgaccatcccatgttggatatagatattttgtggcgtggtactgaatctatcacattaactcgtgatggtttgttaagagctgctatgccaaaacccattggtgattgtgtcttcgtcaatgacctgacaagagaagaattagcagccgcattagctgaccacaaagaactttgtaccagttatccccgtggtggtgaaggtgtggatgtgtatcccgtttatcaaaaagaattaatcgggagtgttaaataatgacttttttgaattcaaaatgcaaaatactccacggatacactgcgcgagcgcggtagcatttctgttcgcggagcgtcccgtagggaaagagaaggctacgcaaataatcggacactaattgtctttaattttgaattttgaattttgaattttgaattggagcgaagcgacttgacaaatgtgattgtccaaccaacagctagacctgttacaccattgggaattttaaccaagcagttagaagccatagtccaagaggttaagcaacatccagatttacctggggaattgatagcaaacatccatcaggcttggcgtttagccgcaggtatagacccttatttggaagaatgcaccactccagaatctcctgaactcgctgcattggcaaaaaccacagccaccgaagcctggggagaacacttccacggaggtacaaccgtccgtcctctagaacaagagatgctttctggtcatatcgaaggacaaaccttaaagatgtttgttcacatgaccaaagctaaaaaagtcttagaaattgggatgtttaccggttattcggcgctggcgatggcggaagcattaccagaggatggactgcttgtggcttgtgaagttgacccttacgcggcggaaattggacagaaagcctttcaacaatctccccacggtggaaagattcgtgtggaattggatgcagccttagcaactcttgataagttagcagaagctggggagtcttttgacttggtatttatcgacgcagataaaaaagagtatgtagcctattttcacaagttgctaggtagcagtttgttagcaccagatggctttatttgtgtagataacaccttattacaaggggaagtttatctaccagcagaggaacgtagcgtcaatggtgaagcgatcgcgcaatttaatcatacagtagctatagacccccgtgtagaacaggttttgttgccgttgcgagatggtttaacaattatccgcagaatacaaccttaa

SEQ ID NO: 86 - protein, 820 aa, Anabaena variabilis ATCC29413
MSIVQAKFEAKETSFHVEGYEKIEYDLVYVDGIFEIQNSALADVYQGFGRCLAIVDANVSRLYGNQIQAYFQYYGIELRLFPITITEPDKTIQTFERVIDVFADFKLVRKEPVLVVGGGLITDVVGFACSTYRRSSNYIRIPTTLIGLIDASVAIKVAVNHRKLKNRLGAYHASRKVFLDFSLLRTLPTDQVRNGMAELVKIAVVAHQEVFELLEKYGEELLRTHFGNIDATPEIKEIAHRLTYKAIHKMLELEVPNLHELDLDRVIAYGHTWSPTLELAPRLPMFHGHAVNVDMAFSATIAARRGYITIAERDRILGLMSRVGLSLDHPMLDIDILWRGTESITLTRDGLLRAAMPKPIGDCVFVNDLTREELAAALADHKELCTSYPRGGEGVDVYPVYQKELIGSVKMSIVQAKFEAKETSFHVEGYEKIEYDLVYVDGIFEIQNSALADVYQGFGRCLAIVDANVSRLYGNQIQAYFQYYGIELRLFPITITEPDKTIQTFERVIDVFADFKLVRKEPVLVVGGGLITDVVGFACSTYRRSSNYIRIPTTLIGLIDASVAIKVAVNHRKLKNRLGAYHASRKVFLDFSLLRTLPTDQVRNGMAELVKIAVVAHQEVFELLEKYGEELLRTHFGNIDATPEIKEIAHRLTYKAIHKMLELEVPNLHELDLDRVIAYGHTWSPTLELAPRLPMFHGHAVNVDMAFSATIAARRGYITIAERDRILGLMSRVGLSLDHPMLDIDILWRGTESITLTRDGLLRAAMPKPIGDCVFVNDLTREELAAALADHKELCTSYPRGGEGVDVYPVYQKELIGSVK

SEQ ID NO: 87 - DNA, 3638 bp, Anabaena variabilis ATCC29413
atgagtatcgtccaagcaaagtttgaagctaaggaaacatcttttcatgtagaaggttacgaaaagattgagtatgatttggtgtatgtagatggtatttttgaaatccagaattctgcactagcagatgtatatcaaggttttggacgatgcttggcgattgtagatgctaacgtcagtcggttgtatggtaatcaaattcaggcatatttccagtattatggtatagaactgaggctatttcctattaccattactgaaccagataagactattcaaactttcgagagagttatagatgtctttgcagatttcaaattagtccgcaaagaaccagtattagtcgtgggtggcggtttaattacagatgttgtcggctttgcttgttctacatatcgtcgcagcagcaattacatccgcattcctactacattgattggattaattgatgccagtgtagcaattaaggtagcagttaatcatcgcaaactgaaaaaccgtttgggtgcttatcatgcttctcgcaaagtatttttagatttctccttgttgcgtactctccctacagaccaagtacgtaacgggatggcggaattggtaaaaatcgctgtagtagcgcatcaagaagtttttgaattgttggagaagtacggcgaagaattactacgtactcattttggcaatatagatgcaactccagagattaaagaaatagcccatcgtttgacttacaaagctatccataagatgttggaattggaagttcccaacctgcatgagttagacctagatagggtgattgcttacggtcacacttggagtcccaccttggaacttgcgcctcgtctacccatgttccacggacacgccgttaatgtagatatggctttctcggcaacgatcgccgcccgtagaggatatattacaattgcagaacgcgatcgtattttaggattaatgagtcgcgttggtctatccctcgaccatcccatgttggatatagatattttgtggcgtggtactgaatctatcacattaactcgtgatggtttgttaagagctgctatgccaaaacccattggtgattgtgtcttcgtcaatgacctgacaagagaagaattagcagccgcattagctgaccacaaagaactttgtaccagttatccccgtggtggtgaaggtgtggatgtgtatcccgtttatcaaaaagaattaatcgggagtgttaaataatgacttttttgaattcaaaatgcaaaatactccacggatacactgcgcgagcgcggtagcatttctgttcgcggagcgtcccgtagggaaagagaaggctacgcaaataatcggacactaattgtctttaattttgaattttgaattttgaattttgaattggagcgaagcgacttgacaaatgtgattgtccaaccaacagctagacctgttacaccattgggaattttaaccaagcagttagaagccatagtccaagaggttaagcaacatccagatttacctggggaattgatagcaaacatccatcaggcttggcgtttagccgcaggtatagacccttatttggaagaatgcaccactccagaatctcctgaactcgctgcattggcaaaaaccacagccaccgaagcctggggagaacacttccacggaggtacaaccgtccgtcctctagaacaagagatgctttctggtcatatcgaaggacaaaccttaaagatgtttgttcacatgaccaaagctaaaaaagtcttagaaattgggatgtttaccggttattcggcgctggcgatggcggaagcattaccagaggatggactgcttgtggcttgtgaagttgacccttacgcggcggaaattggacagaaagcctttcaacaatctccccacggtggaaagattcgtgtggaattggatgcagccttagcaactcttgataagttagcagaagctggggagtcttttgacttggtatttatcgacgcagataaaaaagagtatgtagcctattttcacaagttgctaggtagcagtttgttagcaccagatggctttatttgtgtagataacaccttattacaaggggaagtttatctaccagcagaggaacgtagcgtcaatggtgaagcgatcgcgcaatttaatcatacagtagctatagacccccgtgtagaacaggttttgttgccgttgcgagatggtttaacaattatccgcagaatacaaccttaattgtccaatcgactatggcacaatcccttcccctttcttccgcacctgctacaccgtctcttccttcccagacgaaaatagccgcaattatccaaaatatctgcactttggctttgttattactagcattgcccattaatgccaccattgtttttatatccttgttagtcttccgaccgcaaaaggtcaaagcagcaaacccccaaaccattcttatcagtggcggtaagatgaccaaagctttacaactagcaaggtcattccacgcggctggacatagagttgtcttggtggaaacccataaatactggttgactggtcatcgtttttcccaagcagtggataagttttacacagtccccgcaccccaggacaatccccaagcttacattcaggctttggtagatatcgtcaaacaagaaaacatcgatgtttatattcccgtcaccagtccagtgggtagctactacgactcattagccaaaccagagttatcccattattgcgaagtgtttcactttgacgcagatattacccaaatgttggatgataaatttgcgttgacacaaaaagcgcgatcgcttggtttatcagtacccaaatcctttaaaattacctcaccagaacaagtcatcaacttcgatttttctggagagacacgtaaatacatcctcaaaagcattccctacgactcagtgcggcggttggacttaaccaaactcccctgtgctactccagaggaaacagcagcattcgtcagaagtttgccaattactcccgaaaaaccgtggattatgcaggaatttatccccggtaaggaattctgcacccatagcaccgttcggaatggggaactcagactgcattgctgttgcgaatcttcagccttccaagttaattatgagaatgtaaataacccgcaaattaccgaatgggtacagcattttgtcaaggaactgaaactgacaggacagatttcctttgactttatccaagccgaagacggaacagtttacgccatcgagtgtaacccccgcacacattcagcaattaccacattttacgaccacccccaggtagcagaagcgtacttgagtcaagcaccgacgactgaaaccatacaaccactaacgacaagcaagcctacctattggacttatcacgaagtttggcgtttaactggtatccgttctttcacccagttgcaaagatggctggggaatatttggcgcgggactgatgcgatttatcagccagatgaccccttaccgtttttgatggtacatcattggcaaattcccctactgttattgaataatttgcgtcgtcttaaaggttggacgcggatagatttcaatattgggaagttggtggaattggggggagattag

SEQ ID NO: 88 - protein, 1099 aa, Anabaena variabilis ATCC29413
MSIVQAKFEAKETSFHVEGYEKIEYDLVYVDGIFEIQNSALADVYQGFGRCLAIVDANVSRLYGNQIQAYFQYYGIELRLFPITITEPDKTIQTFERVIDVFADFKLVRKEPVLVVGGGLITDVVGFACSTYRRSSNYIRIPTTLIGLIDASVAIKVAVNHRKLKNRLGAYHASRKVFLDFSLLRTLPTDQVRNGMAELVKIAVVAHQEVFELLEKYGEELLRTHFGNIDATPEIKEIAHRLTYKAIHKMLELEVPNLHELDLDRVIAYGHTWSPTLELAPRLPMFHGHAVNVDMAFSATIAARRGYITIAERDRILGLMSRVGLSLDHPMLDIDILWRGTESITLTRDGLLRAAMPKPIGDCVFVNDLTREELAAALADHKELCTSYPRGGEGVDVYPVYQKELIGSVKMSIVQAKFEAKETSFHVEGYEKIEYDLVYVDGIFEIQNSALADVYQGFGRCLAIVDANVSRLYGNQIQAYFQYYGIELRLFPITITEPDKTIQTFERVIDVFADFKLVRKEPVLVVGGGLITDVVGFACSTYRRSSNYIRIPTTLIGLIDASVAIKVAVNHRKLKNRLGAYHASRKVFLDFSLLRTLPTDQVRNGMAELVKIAVVAHQEVFELLEKYGEELLRTHFGNIDATPEIKEIAHRLTYKAIHKMLELEVPNLHELDLDRVIAYGHTWSPTLELAPRLPMFHGHAVNVDMAFSATIAARRGYITIAERDRILGLMSRVGLSLDHPMLDIDILWRGTESITLTRDGLLRAAMPKPIGDCVFVNDLTREELAAALADHKELCTSYPRGGEGVDVYPVYQKELIGSVKMTNVIVQPTARPVTPLGILTKQLEAIVQEVKQHPDLPGELIANIHQAWRLAAGIDPYLEECTTPESPELAALAKTTATEAWGEHFHGGTTVRPLEQEMLSGHIEGQTLKMFVHMTKAKKVLEIGMFTGYSALAMAEALPEDGLLVACEVDPYAAEIGQKAFQQSPHGGKIRVELDAALATLDKLAEAGESFDLVFIDADKKEYVAYFHKLLGSSLLAPDGFICVDNTLLQGEVYLPAEERSVNGEAIAQFNHTVAIDPRVEQVLLPLRDGLTIIRRIQP

SEQ ID NO: 89 - DNA, 1233 bp, Anabaena variabilis ATCC29413
atgagtatcgtccaagcaaagtttgaagctaaggaaacatcttttcatgtagaaggttacgaaaagattgagtatgatttggtgtatgtagatggtatttttgaaatccagaattctgcactagcagatgtatatcaaggttttggacgatgcttggcgattgtagatgctaacgtcagtcggttgtatggtaatcaaattcaggcatatttccagtattatggtatagaactgaggctatttcctattaccattactgaaccagataagactattcaaactttcgagagagttatagatgtctttgcagatttcaaattagtccgcaaagaaccagtattagtcgtgggtggcggtttaattacagatgttgtcggctttgcttgttctacatatcgtcgcagcagcaattacatccgcattcctactacattgattggattaattgatgccagtgtagcaattaaggtagcagttaatcatcgcaaactgaaaaaccgtttgggtgcttatcatgcttctcgcaaagtatttttagatttctccttgttgcgtactctccctacagaccaagtacgtaacgggatggcggaattggtaaaaatcgctgtagtagcgcatcaagaagtttttgaattgttggagaagtacggcgaagaattactacgtactcattttggcaatatagatgcaactccagagattaaagaaatagcccatcgtttgacttacaaagctatccataagatgttggaattggaagttcccaacctgcatgagttagacctagatagggtgattgcttacggtcacacttggagtcccaccttggaacttgcgcctcgtctacccatgttccacggacacgccgttaatgtagatatggctttctcggcaacgatcgccgcccgtagaggatatattacaattgcagaacgcgatcgtattttaggattaatgagtcgcgttggtctatccctcgaccatcccatgttggatatagatattttgtggcgtggtactgaatctatcacattaactcgtgatggtttgttaagagctgctatgccaaaacccattggtgattgtgtcttcgtcaatgacctgacaagagaagaattagcagccgcattagctgaccacaaagaactttgtaccagttatccccgtggtggtgaaggtgtggatgtgtatcccgtttatcaaaaagaattaatcgggagtgttaaataa

SEQ ID NO: 90 - protein, 410 aa, Anabaena variabilis ATCC29413
MSIVQAKFEAKETSFHVEGYEKIEYDLVYVDGIFEIQNSALADVYQGFGRCLAIVDANVSRLYGNQIQAYFQYYGIELRLFPITITEPDKTIQTFERVIDVFADFKLVRKEPVLVVGGGLITDVVGFACSTYRRSSNYIRIPTTLIGLIDASVAIKVAVNHRKLKNRLGAYHASRKVFLDFSLLRTLPTDQVRNGMAELVKIAVVAHQEVFELLEKYGEELLRTHFGNIDATPEIKEIAHRLTYKAIHKMLELEVPNLHELDLDRVIAYGHTWSPTLELAPRLPMFHGHAVNVDMAFSATIAARRGYITIAERDRILGLMSRVGLSLDHPMLDIDILWRGTESITLTRDGLLRAAMPKPIGDCVFVNDLTREELAAALADHKELCTSYPRGGEGVDVYPVYQKELIGSVK

SEQ ID NO: 91 - DNA, 840 bp, Anabaena variabilis ATCC29413
ttgacaaatgtgattgtccaaccaacagctagacctgttacaccattgggaattttaaccaagcagttagaagccatagtccaagaggttaagcaacatccagatttacctggggaattgatagcaaacatccatcaggcttggcgtttagccgcaggtatagacccttatttggaagaatgcaccactccagaatctcctgaactcgctgcattggcaaaaaccacagccaccgaagcctggggagaacacttccacggaggtacaaccgtccgtcctctagaacaagagatgctttctggtcatatcgaaggacaaaccttaaagatgtttgttcacatgaccaaagctaaaaaagtcttagaaattgggatgtttaccggttattcggcgctggcgatggcggaagcattaccagaggatggactgcttgtggcttgtgaagttgacccttacgcggcggaaattggacagaaagcctttcaacaatctccccacggtggaaagattcgtgtggaattggatgcagccttagcaactcttgataagttagcagaagctggggagtcttttgacttggtatttatcgacgcagataaaaaagagtatgtagcctattttcacaagttgctaggtagcagtttgttagcaccagatggctttatttgtgtagataacaccttattacaaggggaagtttatctaccagcagaggaacgtagcgtcaatggtgaagcgatcgcgcaatttaatcatacagtagctatagacccccgtgtagaacaggttttgttgccgttgcgagatggtttaacaattatccgcagaatacaaccttaa

SEQ ID NO: 92 - protein, 410 aa, Anabaena variabilis ATCC29413; identical to SEQ ID NO: 90

SEQ ID NO: 93 - DNA, 840 bp, Anabaena variabilis ATCC29413; identical to SEQ ID NO: 91

SEQ ID NO: 94 - protein, 279 aa, Anabaena variabilis ATCC29413
MTNVIVQPTARPVTPLGILTKQLEAIVQEVKQHPDLPGELIANIHQAWRLAAGIDPYLEECTTPESPELAALAKTTATEAWGEHFHGGTTVRPLEQEMLSGHIEGQTLKMFVHMTKAKKVLEIGMFTGYSALAMAEALPEDGLLVACEVDPYAAEIGQKAFQQSPHGGKIRVELDAALATLDKLAEAGESFDLVFIDADKKEYVAYFHKLLGSSLLAPDGFICVDNTLLQGEVYLPAEERSVNGEAIAQFNHTVAIDPRVEQVLLPLRDGLTIIRRIQP

SEQ ID NO: 95 - DNA, 2667 bp, Anabaena variabilis ATCC29413
atgcagactatagattttaatattcgtaagttacttgtagagtggaacgcgacccacagagattatgatctttcccagagtttacatgaactaattgtagctcaagtagaacgaacacctgaggcgatcgctgtcacctttgacaagcaacaactaacttatcaagaactaaatcataaagcaaaccagctaggacattatttacaaacattaggagtccagccagaaaccctggtaggcgtttgtttagaacgttccttagaaatggttatctgtcttttaggaatcctcaaagctgggggtgcttatgttcctattgaccctgaatatcctcaagaacgcatagcttatatgctagaagattctcaggtgaaggtactactaactcaagaaaaattactcaatcaaattccccaccatcaagcacaaactatctgtgtagatagggaatgggagaaaatttccacacaagctaataccaatcccaaaagtaatataaaaacggataatcttgcttatgtaatttacacctctggttccactggtaaaccaaaaggtgcaatgaacacccacaaaggtatctgtaatcgcttattgtggatgcaggaagcttatcaaatcgattccacagatagcattttacaaaaaaccccctttagttttgatgtttccgtttgggagttcttttggactttattaactggcgcacgtttggtaatagccaaaccaggcggacataaagatagtgcttacctcatcgatttaattactcaagaacaaatcactacgttgcattttgtcccctcaatgctgcaagtgtttttacaaaatcgccatgtaagcaaatgcagctctctaaaaagagttatttgtagcggtgaagctttatctatagatttacaaaatagatttttccagcatttgcaatgtgaattacataacctctatggcccgacagaagcagcaattgatgtcacattttggcaatgtagaaaagatagtaatttaaagagtgtacctattggtcgtcccattgctaatactcaaatttatattcttgatgccgatttacaaccagtaaatattggtgtcactggtgaaatttatattggtggtgtaggggttgctcgtggttatttgaataaagaagaattgaccaaagaaaaatttattattaatccctttcccaattctgagtttaagcgactttataaaacaggtgatttagctcgttatttacccgatggaaatattgaatatcttggtagaacagattatcaagtaaaaattcggggttatagaattgaaattggcgagattgaaaatgttttatcttcacacccacaagtcagagaagctgtagtcatagcgcgggatgataacgctcaagaaaaacaaatcatcgcttatattacctataactccatcaaacctcagcttgataatctgcgtgatttcctaaaagcaaggctacctgattttatgattccagccgcttttgtgatgctggagcatcttcctttaactcccagtggtaaagtagaccgtaaggcattacctaagcctgatttatttaattatagtgaacataattcctatgtagcgcctcggaatgaagttgaagaaaaattagtacaaatctggtcgaatattctgcatttacctaaagtaggtgtgacagaaaactttttcgctattggtggtaattccctcaaagctctacatttaatttctcaaattgaagagttatttgctaaagagatatccttagcaacacttttaacaaatccagtaattgcagatttagccaaggttattcaagcaaacaaccaaatccataattcacccctagttccaattcaaccacaaggtaagcagcagcctttcttttgtatacatcctgctggtggtcatgttttatgctattttaaactcgcacaatatataggaactgaccaaccattttatggcttacaagctcaaggattttatggagatgaagcacccttgacgcgagttgaagatatggctagtctctacgtcaaaactattagagaatttcaaccccaagggccttatcgtgtcggggggtggtcatttggtggagtcgtagcttatgaagtagcacagcagttacatagacaaggacaagaagtatctttactagcaatattagattcttacgtaccgattctgctggataaacaaaaacccattgatgacgtttatttagttggtgttctctccagagtttttggcggtatgtttggtcaagataatctagtcacacctgaagaaatagaaaatttaactgtagaagaaaaaattaattacatcattgataaagcacggagcgctagaatattcccgcctggtgtagaacgtcaaaataatcgccgtattcttgatgttttggtgggaactttaaaagcaacttattcctatataagacaaccatatccaggaaaagtcactgtatttcgagccagggaaaaacatattatggctcctgacccgaccttagtttgggtagaattattttctgtaatggcggctcaagaaattaagattattgatgtccctggaaaccattattcgtttgttctagaaccccatgtacaggttttagcacagcgtttacaagattgtctggaaaataattcataa

SEQ ID NO: 96 - protein, 888 aa, Anabaena variabilis ATCC29413
MQTIDFNIRKLLVEWNATHRDYDLSQSLHELIVAQVERTPEAIAVTFDKQQLTYQELNHKANQLGHYLQTLGVQPETLVGVCLERSLEMVICLLGILKAGGAYVPIDPEYPQERIAYMLEDSQVKVLLTQEKLLNQIPHHQAQTICVDREWEKISTQANTNPKSNIKTDNLAYVIYTSGSTGKPKGAMNTHKGICNRLLWMQEAYQIDSTDSILQKTPFSFDVSVWEFFWTLLTGARLVIAKPGGHKDSAYLIDLITQEQITTLHFVPSMLQVFLQNRHVSKCSSLKRVICSGEALSIDLQNRFFQHLQCELHNLYGPTEAAIDVTFWQCRKDSNLKSVPIGRPIANTQIYILDADLQPVNIGVTGEIYIGGVGVARGYLNKEELTKEKFIINPFPNSEFKRLYKTGDLARYLPDGNIEYLGRTDYQVKIRGYRIEIGEIENVLSSHPQVREAVVIARDDNAQEKQIIAYITYNSIKPQLDNLRDFLKARLPDFMIPAAFVMLEHLPLTPSGKVDRKALPKPDLFNYSEHNSYVAPRNEVEEKLVQIWSNILHLPKVGVTENFFAIGGNSLKALHLISQIEELFAKEISLATLLTNPVIADLAKVIQANNQIHNSPLVPIQPQGKQQPFFCIHPAGGHVLCYFKLAQYIGTDQPFYGLQAQGFYGDEAPLTRVEDMASLYVKTIREFQPQGPYRVGGWSFGGVVAYEVAQQLHRQGQEVSLLAILDSYVPILLDKQKPIDDVYLVGVLSRVFGGMFGQDNLVTPEEIENLTVEEKINYIIDKARSARIFPPGVERQNNRRILDVLVGTLKATYSYIRQPYPGKVTVFRAREKHIMAPDPTLVWVELFSVMAAQEIKIIDVPGNHYSFVLEPHVQVLAQRLQDCLENNS

SEQ ID NO: 97 - DNA, 1233 bp, Nostoc punctiforme ATCC29133
atgagtaatgttcaagcatcgtttgaagcaacggaagctgaattccgcgtggaaggttacgaaaaaattgagtttagtcttgtctatgtaaatggtgcatttgatatcagtaacagagaaattgcagacagctatgagaagtttggccgttgtctgactgtgattgatgctaatgtcaacagattatatggcaagcaaatcaagtcatattttagacactatggtattgatctgaccgtagttcccattgtgattactgagcctactaaaacccttgcaacctttgagaaaattgttgatgctttttctgactttggtttaatccgcaaggaaccagtattagtagtgggtggtggtttaaccactgatgtagctgggtttgcgtgtgctgcttaccgtcgtaagagtaactatattcgggttccgacaacgctgattggtctgattgatgcaggtgtagcgattaaggttgcagtcaaccatcgcaagttaaaaaatcgcttgggtgcatatcatgctcctttgaaagtcatcctcgatttctccttcttgcaaacattaccaacggctcaagttcgtaatgggatggcagagttggtcaaaattgctgttgtggcgaactctgaagtctttgaattgttgtatgaatatggcgaagagttgctttccactcactttggatatgtgaatggtacaaaggaactgaaagcgatcgcacataaactcaattacgaggcaataaaaactatgctggagttggaaactccaaacttgcatgagttagacctcgatcgcgtcattgcctacggtcacacttggagtccgaccttagaattagctccgatgataccgttgtttcacggtcatgccgtcaatatagacatggctttgtctgcaactattgcggcaagacgtggctacattacatcaggagaacgcgatcgcattttgagcttgatgagtcgtataggtttatcaatcgatcatcctctactagatggcgatttgctctggtatgctacccaatctattagcttgacgcgagacgggaaacaacgcgcagctatgcctaaacccattggtgagtgcttctttgtcaacgatttcacccgtgaagaactagatgcagctttagctgaacacaaacgtctgtgtgctacataccctcgtggtggagatggcattgacgcttacatagaaactcaagaagaatccaaactattgggagtgtga

SEQ ID NO: 98 - protein, 410 aa, Nostoc punctiforme ATCC29133
MSNVQASFEATEAEFRVEGYEKIEFSLVYVNGAFDISNREIADSYEKFGRCLTVIDANVNRLYGKQIKSYFRHYGIDLTVVPIVITEPTKTLATFEKIVDAFSDFGLIRKEPVLVVGGGLTTDVAGFACAAYRRKSNYIRVPTTLIGLIDAGVAIKVAVNHRKLKNRLGAYHAPLKVILDFSFLQTLPTAQVRNGMAELVKIAVVANSEVFELLYEYGEELLSTHFGYVNGTKELKAIAHKLNYEAIKTMLELETPNLHELDLDRVIAYGHTWSPTLELAPMIPLFHGHAVNIDMALSATIAARRGYITSGERDRILSLMSRIGLSIDHPLLDGDLLWYATQSISLTRDGKQRAAMPKPIGECFFVNDFTREELDAALAEHKRLCATYPRGGDGIDAYIETQEESKLLGV

SEQ ID NO: 99 - DNA, 834 bp, Nostoc punctiforme ATCC29133
atgaccagtattttaggacgagataccgcaagaccaataacgccacatagcattctggtagcacagctacaaaaaaccctcagaatggcagaggaaagtaatattccttcagagatactgacttctctgcgccaagggttgcaattagcagcaggtttagatccctatctggatgattgcactacccctgaatcgaccgcattgacagcactagcgcagaagacaagcattgaagactggagtaaacgcttcagtgatggtgaaacagtgcgtcaattagagcaagaaatgctctcaggacatcttgaaggacaaacactaaagatgtttgtgcatatcactaaggctaaaagcatcctagaagtgggaatgttcacaggatattcagctttggcaatggcagaggcgttaccagatgatgggcgactgattgcttgtgaagtagactcctatgtggccgagtttgctcaaacttgctttcaagagtctccccacggccgcaagattgttgtagaagtggcacctgcactagagacgctgcacaagctggtggctaaaaaagaatcctttgatctgatcttcattgatgcggataaaaaggagtatatagaatacttccaaattatcttggatagccatttactagctcccgacggattaatctgtgtagataatactttgttgcaaggacaagtttacctgccatcagaacagcgtacagccaatggtgaagcgatcgctcaattcaaccgcattgtcgccgcagatcctcgtgtagagcaagttctgttacccatacgagatggtataaccctgattagacgcttggtataa

SEQ ID NO: 100 - protein, 277 aa, Nostoc punctiforme ATCC29133
MTSILGRDTARPITPHSILVAQLQKTLRMAEESNIPSEILTSLRQGLQLAAGLDPYLDDCTTPESTALTALAQKTSIEDWSKRFSDGETVRQLEQEMLSGHLEGQTLKMFVHITKAKSILEVGMFTGYSALAMAEALPDDGRLIACEVDSYVAEFAQTCFQESPHGRKIVVEVAPALETLHKLVAKKESFDLIFIDADKKEYIEYFQIILDSHLLAPDGLICVDNTLLQGQVYLPSEQRTANGEAIAQFNRIVAADPRVEQVLLPIRDGITLIRRLV

SEQ ID NO: 101 - DNA, 1386 bp, Nostoc punctiforme ATCC29133
atggcacaatcaatctctttatctcttcctcaatccacaacgccatcaaagggtgtgaggctaaaaatagcagctctactgaagactatcgggactctaatactactgctgatagccttgccgcttaatgctttgatagtattgatatctctgatgtgtaggccgtttacaaaaaaacctgccgtagccactcatccccagaatatcttggtcagtggcggcaaaatgaccaaagcattgcaacttgcccgctccttccatgcagccggacacagagttattctgattgaaggtcataaatactggttatcagggcatagattctcaaattctgtgagtcgtttttatacagttcctgcaccacaagacgacccagaaggctatacccaagcgctattggaaattgtcaaacgagagaagattgacgtttatgtacccgtatgcagccctgtagctagttattacgactctttggcaaagtctgcactatcagaatattgtgaggtttttcactttgatgctgatataaccaagatgctggatgataaatttgcctttaccgatcgggcgcgatcgcttggtttatcagccccgaaatcttttaaaattaccgatcctgaacaagttatcaacttcgattttagtaaagagacgcgcaaatatattcttaagagtatttcttacgactcagttcgccgcttaaatttaaccaaacttccttgtgataccccagaagagacagcagcgtttgtcaagagtttacccatcagcccagaaaaaccttggattatgcaagaatttattcctgggaaagaattatgcacccatagcacagtccgagacggcgaattaaggttgcattgctgttcaaattcttcagcgtttcagattaactatgaaaatgtcgaaaatccccaaattcaagaatgggtacaacatttcgtcaaaagtttacggctgactggacaaatatctcttgactttatccaagctgaagatggtacagcttatgccattgaatgtaatcctcgcacccattcggcgatcacaatgttctacaatcacccaggtgttgcagaagcctatcttggtaaaactcctctagctgcacctttggaacctcttgcagatagcaagcccacttactggatatatcacgaaatctggcgattgactgggattcgctctggacaacaattacaaacttggtttgggagattagtcagaggtacagatgccatttatcgcctggacgatccgataccatttttaactttgcaccattggcagattactttacttttgctacaaaatttgcaacgactcaaaggttgggtaaagatcgattttaatatcggtaaactcgtggaattagggggcgactaa

SEQ ID NO: 102 - protein, 461 aa, Nostoc punctiforme ATCC29133
MAQSISLSLPQSTTPSKGVRLKIAALLKTIGTLILLLIALPLNALIVLISLMCRPFTKKPAVATHPQNILVSGGKMTKALQLARSFHAAGHRVILIEGHKYWLSGHRFSNSVSRFYTVPAPQDDPEGYTQALLEIVKREKIDVYVPVCSPVASYYDSLAKSALSEYCEVFHFDADITKMLDDKFAFTDRARSLGLSAPKSFKITDPEQVINFDFSKETRKYILKSISYDSVRRLNLTKLPCDTPEETAAFVKSLPISPEKPWIMQEFIPGKELCTHSTVRDGELRLHCCSNSSAFQINYENVENPQIQEWVQHFVKSLRLTGQISLDFIQAEDGTAYAIECNPRTHSAITMFYNHPGVAEAYLGKTPLAAPLEPLADSKPTYWIYHEIWRLTGIRSGQQLQTWFGRLVRGTDAIYRLDDPIPFLTLHHWQITLLLLQNLQRLKGWVKIDFNIGKLVELGGD

SEQ ID NO: 103 - DNA, 1047 bp, Nostoc punctiforme ATCC29133
atgccagtacttaatatccttcatttagttgggtctgcacacgataagttttactgtgatttatcacgtctttatgcccaagactgtttagctgcaacagcagatccatcgctttataactttcaaattgcatatatcacacccgatcggcagtggcgatttcctgactctctcagtcgagaagatattgctcttaccaaaccgattcctgtgtttgatgccatacaatttctaacaggccaaaacattgacatgatgttaccacaaatgttttgtattcctggaatgactcagtaccgtgccctattcgatctgctcaagatcccttatataggaaataccccagatattatggcgatcgcggcccacaaagccagagccaaagcaattgtcgaagcagcaggggtaaaagtgcctcgtggagaattgcttcgccaaggagatattccaacaattacacctccagcagtcgtcaaacctgtaagttctgacaactctttaggagtagtcttagttaaagatgtgactgaatatgatgctgccttaaagaaagcatttgaatatgcttcggaggtcatcgtagaagcattcatcgaacttggtcgagaagtcagatgcggcatcattgtaaaagacggtgagctaataggtttaccccttgaagagtatctggtagacccacacgataaacctatccgtaactatgctgataaactccaacaaactgacgatggcgacttgcatttgactgctaaagataatatcaaggcttggattttagaccctaacgacccaatcacccaaaaggttcagcaagtggctaaaaggtgtcatcaggctttgggttgtcgccactacagtttatttgacttccgaatcgatccaaagggacaaccttggttcttagaagctggattatattgttcttttgcccccaaaagtgtgatttcttctatggcgaaagcagccggaatccctctaaatgatttattaataaccgctattaatgaaacattgggtagtaataaaaaggtgttacaaaattga

SEQ ID NO: 104 - protein, 348 aa, Nostoc punctiforme ATCC29133
MPVLNILHLVGSAHDKFYCDLSRLYAQDCLAATADPSLYNFQIAYITPDRQWRFPDSLSREDIALTKPIPVFDAIQFLTGQNIDMMLPQMFCIPGMTQYRALFDLLKIPYIGNTPDIMAIAAHKARAKAIVEAAGVKVPRGELLRQGDIPTITPPAVVKPVSSDNSLGVVLVKDVTEYDAALKKAFEYASEVIVEAFIELGREVRCGIIVKDGELIGLPLEEYLVDPHDKPIRNYADKLQQTDDGDLHLTAKDNIKAWILDPNDPITQKVQQVAKRCHQALGCRHYSLFDFRIDPKGQPWFLEAGLYCSFAPKSVISSMAKAAGIPLNDLLITAINETLGSNKKVLQN